European Patent Specification EP 3 864 177 B1, published February 25, 2026. Title: DNA METHYLATION BASED BIOMARKERS FOR LIFE EXPECTANCY AND MORBIDITY. Applicant: UNIVERSITY OF CALIFORNIA. The sequence listing filed with the application follows.

SEQUENCE LISTING (1113 sequences)

SEQ ID NO: 1 - DNA, 50 bp, Homo sapiens
cgggaccgtttggccctctgtgacccaagtcagcctcggcgaagtgcttt

SEQ ID NO: 2 - DNA, 50 bp, Homo sapiens
cgcggccaggcagcgaaccccactaggaggcaccccaggcccctgggctt

SEQ ID NO: 3 - DNA, 50 bp, Homo sapiens
cgcgcctgggcccccaggacctcttgcagacgggagtccctcagacagtg

SEQ ID NO: 4 - DNA, 50 bp, Homo sapiens
ggttgcttccttttgtgccccccgggggtcaggaatcccaggtttctccg

SEQ ID NO: 5 - DNA, 50 bp, Homo sapiens
ctgaggccacctggggctggggatcccactcttcttgcagctgttgagcg

SEQ ID NO: 6 - DNA, 50 bp, Homo sapiens
agggccccctgggcctgtaccaaggtctgcgacagatgggtggggagccg

SEQ ID NO: 7 - DNA, 50 bp, Homo sapiens
gcctggcagaatcaggagccgggggagtagggctcccggaaagtttatcg

SEQ ID NO: 8 - DNA, 50 bp, Homo sapiens
gaggcagtgggcggggctgaagctgcaggtctggcagagggcgggctgcg

SEQ ID NO: 9 - DNA, 50 bp, Homo sapiens
gtgggcggggctgaagctgcaggtctggcagagggcgggctgcggcagcg

SEQ ID NO: 10 - DNA, 50 bp, Homo sapiens
cgcaagcatgaagcgtttaactgtgcaacacaaatcaacaacctgggctc

SEQ ID NO: 11 - DNA, 50 bp, Homo sapiens
cgcacccactgaatcagaagctgtaggagcgggagccagtggtttgcatt

SEQ ID NO: 12 - DNA, 50 bp, Homo sapiens
cgctgccaaacccctacacgaaagtttggttctgttccagaaactatgga

SEQ ID NO: 13 - DNA, 50 bp, Homo sapiens
ggacaaaaatcctcggtggcgggggcaaaaagtcgcggtgacaaaaagcg

SEQ ID NO: 14 - DNA, 50 bp, Homo sapiens
tttgaagcccttatgtctatggtaatctgttacagcccccgcaggaaacg

SEQ ID NO: 15 - DNA, 50 bp, Homo sapiens
cgggcaccttgctgctggccctcggccccacgcacctgcccttggctgcc

SEQ ID NO: 16 - DNA, 50 bp, Homo sapiens
cgtgaattgagatgtcatgccattgtaagatttttaaaaagggaaggaca

SEQ ID NO: 17 - DNA, 50 bp, Homo sapiens
cggcgcgcactgcacaatgaacatgcaaaacaccttcaactgcacttgct

SEQ ID NO: 18 - DNA, 50 bp, Homo sapiens
ccatagcggtgggcctttggcgacgtcagaggcgcgggtgttcgcctacg

SEQ ID NO: 19 - DNA, 50 bp, Homo sapiens
agctcctgccgtggtggtgaaatattgtggactgcttggctgactacacg

SEQ ID NO: 20 - DNA, 50 bp, Homo sapiens
cgtgctcagctgataaaatgctaaatagcatcaatgctgaccatgcttct

SEQ ID NO: 21 - DNA, 50 bp, Homo sapiens
cgtgtgtacacatgtatgtctttcaagcaaggctatgtattactcagaac

SEQ ID NO: 22 - DNA, 50 bp, Homo sapiens
gtcagggagataagtccctttgcggaatgtcaagacggtgagcaggcgcg

SEQ ID NO: 23 - DNA, 50 bp, Homo sapiens
cgcttcttaagggaaaggcatgaggtgggacaggcaaaccttggcaagtg

SEQ ID NO: 24 - DNA, 50 bp, Homo sapiens
cggcaggcatcccctctacctgaccggcttcttcggaggatacatcttgg

SEQ ID NO: 25 - DNA, 50 bp, Homo sapiens
attagcggagcctccgcctatgattggcttcgcccgggaagctggagacg

SEQ ID NO: 26 - DNA, 50 bp, Homo sapiens
cgggggctcttcctgctcaagctgggacttagcctgctcatgttgttggc

SEQ ID NO: 27 - DNA, 50 bp, Homo sapiens
ctttttttggcattggaattggcaagtggctgcccttgtctgttacaacg

SEQ ID NO: 28 - DNA, 50 bp, Homo sapiens
cggggtgcaggtcagggctccaggtgtcacctgcctgtccacacggggct

SEQ ID NO: 29 - DNA, 50 bp, Homo sapiens
cgccgtgtccctcacgctggctttcagaaggcttcacgcaagtgggctca

SEQ ID NO: 30 - DNA, 50 bp, Homo sapiens
cgggtgctgttatcaccccaatttcaccaatgaggaaagaggtgcagaga

SEQ ID NO: 31 - DNA, 50 bp, Homo sapiens
gtggttttctacctggacctctccttcatcttcctcctagaactgaagcg

SEQ ID NO: 32 - DNA, 50 bp, Homo sapiens
gctgtggcgtctccaactacactgactggttcgaggtgtacaacgccacg

SEQ ID NO: 33 - DNA, 50 bp, Homo sapiens
cgtggacttcccatcccctggaccccacggcggggacaaggaaacctaca

SEQ ID NO: 34 - DNA, 50 bp, Homo sapiens
agcctcactgaggaagtgactgtcccaggctctagaggtgcctgagggcg

SEQ ID NO: 35 - DNA, 50 bp, Homo sapiens
agacggggaggccgggcagagacgctcctcacctcccagacagggttgcg

SEQ ID NO: 36 - DNA, 50 bp, Homo sapiens
cgaccctttgtggagggcactggaggagctggcatttaagccctgtccag

SEQ ID NO: 37 - DNA, 50 bp, Homo sapiens
aatgcgtcgcagtcaagacagcgcaggggcctgggctgccgggcgctgcg

SEQ ID NO: 38 - DNA, 50 bp, Homo sapiens
caagggcacacagcgaggcagtttcagggcgggcagcctggggccccacg

SEQ ID NO: 39 - DNA, 50 bp, Homo sapiens
cggggcagtgctttcccagaaggattgctcggcatcctgcccttcccaga

SEQ ID NO: 40 - DNA, 50 bp, Homo sapiens
cgcacagcactgagtgctgtaaggaaatgcaaagcattggtggccctgcc

SEQ ID NO: 41 - DNA, 50 bp, Homo sapiens
cggtgcctccaaagaacagaaacctgtattcccatggcagggccaccaat

SEQ ID NO: 42 - DNA, 50 bp, Homo sapiens
tctcaaactcggggccagagaacagtgaagtaggagcagccgtaagtccg

SEQ ID NO: 43 - DNA, 50 bp, Homo sapiens
cgccccggcccgctccatctccaaagcatgcagagaatgtctcggcagcc

SEQ ID NO: 44 - DNA, 50 bp, Homo sapiens
gcacacacagcagcagcactgccacccagagcagggctaagatgaacacg

SEQ ID NO: 45 - DNA, 50 bp, Homo sapiens
cgggtattactgccatcgtcgtaccagcagggaaacaaactgagactccg

SEQ ID NO: 46 - DNA, 50 bp, Homo sapiens
cgcggctccatactattgcccagtgttttccgagcatctccatccttggc

SEQ ID NO: 47 - DNA, 50 bp, Homo sapiens
cagtccgtcatctcatctggggaaactgtttgcctttttctgatactacg

SEQ ID NO: 48 - DNA, 50 bp, Homo sapiens
cgtgtgcacatgcgcactctcatatgccaccccatgtgcctttagtccac

SEQ ID NO: 49 - DNA, 50 bp, Homo sapiens
caggagatgccgcggtagggggcggcggtgatgcagcagcggcttggccg

SEQ ID NO: 50 - DNA, 50 bp, Homo sapiens
cgggtgcccaggagcccacaaaacggccagaggagaaatgctttcaaagg

SEQ ID NO: 51 - DNA, 50 bp, Homo sapiens
cggccttctggctggcaagcccctgtgggccaggaagctcagacctaacc

SEQ ID NO: 52 - DNA, 50 bp, Homo sapiens
agtcactgaatcatgagtgacggtaacataaatgcccatcgggggaaacg

SEQ ID NO: 53 - DNA, 50 bp, Homo sapiens
actcgccttgatgttcattggggttcaaaataatcaagttctgcagaacg

SEQ ID NO: 54 - DNA, 50 bp, Homo sapiens
ggccaaggcaggcggctgggaggcgtaggttgtagcgagccgagatcacg

SEQ ID NO: 55 - DNA, 50 bp, Homo sapiens
acgatgttggctcactgcatcctccaccttctgggttcaagcgattctcg

SEQ ID NO: 56 - DNA, 50 bp, Homo sapiens
gtcatccccggggagaggctctcaatggggagtcccatctgcaggctgcg

SEQ ID NO: 57 - DNA, 50 bp, Homo sapiens
cgggttccttttaaagtgctgctagcgcgcactcgccctctcagcgttgc

SEQ ID NO: 58 - DNA, 50 bp, Homo sapiens
caaggccactgcaatttttgggatctagtgagtctgtaggaaatgtaacg

SEQ ID NO: 59 - DNA, 50 bp, Homo sapiens
tgaggtcaggcgtgcccttgcgtagcacaatcgcggggaggggtggctcg

SEQ ID NO: 60 - DNA, 50 bp, Homo sapiens
gcatgtggcatgggtggggtggccagcacgctacaggggcttcctatgcg

SEQ ID NO: 61 - DNA, 50 bp, Homo sapiens
cggaagaggctccagtgtcctcagcagacatgctttatttggttaaagca

SEQ ID NO: 62 - DNA, 50 bp, Homo sapiens
aagcttcagtgaatgtcccccgcttctaagatcctcttctttttgtcacg

SEQ ID NO: 63 - DNA, 50 bp, Homo sapiens
cgccaggctcgcgatgcctctacacaagtatcccgtgtggctctggaagc

SEQ ID NO: 64 - DNA, 50 bp, Homo sapiens
cgggagaaccttctgtgcaggcccggcgctgctccactccaggaaagaaa

SEQ ID NO: 65 - DNA, 50 bp, Homo sapiens
gaggcagggcaggcagacctgcagtcactcctctgcagagtcgcacaccg

SEQ ID NO: 66 - DNA, 50 bp, Homo sapiens
cgcagagaaggaaataacttgttcaaaagaacctactggggtgtgtgtac

SEQ ID NO: 67 - DNA, 50 bp, Homo sapiens
gggagtgggctggcagtgcgcgcacagcggcggcgagtgggtcgtgcacg

SEQ ID NO: 68 - DNA, 50 bp, Homo sapiens
tcgttcctcatgaaaacatcttgagtccaggatctccaattgcactcacg

SEQ ID NO: 69 - DNA, 50 bp, Homo sapiens
ttctctcaaaactcatcacccacttttctttaactgtttgttataagacg

SEQ ID NO: 70 - DNA, 50 bp, Homo sapiens
cggacctagactccaacagtgacagctctgagtaaagaagtcgccgaagc

SEQ ID NO: 71 - DNA, 50 bp, Homo sapiens
gaaggagaagcacccggagccggggggctcctgtgtctactgcaaaagcg

SEQ ID NO: 72 - DNA, 50 bp, Homo sapiens
tggccgggatcccgtgcttggcatacagccggtcttgttctcattgtccg

SEQ ID NO: 73 - DNA, 50 bp, Homo sapiens
ttcatgggtgtggtagcttgtgagaccggccggctgcgcccatgcccccg

SEQ ID NO: 74 - DNA, 50 bp, Homo sapiens
tttaacctttccaggcctcagtttcttcatctgttcagtggaaatgatcg

SEQ ID NO: 75 - DNA, 50 bp, Homo sapiens
tagttttcaccaccctgcctggagcagcacagccaatattggcagactcg

SEQ ID NO: 76 - DNA, 50 bp, Homo sapiens
cgcaagccggccctcacccagtatattgatagggccattgaggggttccg

SEQ ID NO: 77 - DNA, 50 bp, Homo sapiens
cggcctgctaaggaacctcaattaatagctcactgtagccttctgattct

SEQ ID NO: 78 - DNA, 50 bp, Homo sapiens
gacccagaggcactggggtagggctcggcagggcgggtccgggcggagcg

SEQ ID NO: 79 - DNA, 50 bp, Homo sapiens
ctgggctccatgtgtaatttcagggctcatggccacacccagcattgacg

SEQ ID NO: 80 - DNA, 50 bp, Homo sapiens
cgggtaagccccgctgtgttctcatacccgaacggcaggaacacaggcag

SEQ ID NO: 81 - DNA, 50 bp, Homo sapiens
cgcacagagccgcacgggactcagtttccacacacacagagccacacggg

SEQ ID NO: 82 - DNA, 50 bp, Homo sapiens
taagaataacttttgcctcctactgtgattctgaggcctccccaatcacg

SEQ ID NO: 83 - DNA, 50 bp, Homo sapiens
gtggtgacagagccacagagggctgtgagcttgcccggccccaggtaacg

SEQ ID NO: 84 - DNA, 50 bp, Homo sapiens
tggtggtggggctgccggccaatgggctggcgctgtgggtgctggccacg

SEQ ID NO: 85 - DNA, 50 bp, Homo sapiens
cggggcgctgagctcaggcccagaactggctgatttcagggatacccagg

SEQ ID NO: 86 - DNA, 50 bp, Homo sapiens
cggcgcagacaccccgttcggacgatcagagagtgccccaaccctacacc

SEQ ID NO: 87 - DNA, 50 bp, Homo sapiens
gatgaccgggatacagtttgctgcattgcaagggctcacccagtgttccg

SEQ ID NO: 88 - DNA, 50 bp, Homo sapiens
gtcaaaggacaagcccctgggacctgcccaatgctggttcaggggaagcg

SEQ ID NO: 89 - DNA, 50 bp, Homo sapiens
cggggcggaatatacgatttcatgctgatggcccacagaacataacagaa

SEQ ID NO: 90 - DNA, 50 bp, Homo sapiens
cgtgtggacgcgggaggaaaccagagtgcccagagacaacccacgcagac

SEQ ID NO: 91 - DNA, 50 bp, Homo sapiens
ccatgcagggctctagacagcggcgctgcagagcttcctgaggtcggccg

SEQ ID NO: 92 - DNA, 50 bp, Homo sapiens
ctagctttagctgcacattagagtcacctgcagctcttttcaaactgtcg

SEQ ID NO: 93 - DNA, 50 bp, Homo sapiens
ggggggtcaatactcacctggtcgtagacaggagccctggagtcggagcg

SEQ ID NO: 94 - DNA, 50 bp, Homo sapiens
cgtgtctcagtgacgctgattctgcttcacaacaaaagcaaaacaagaac

SEQ ID NO: 95 - DNA, 50 bp, Homo sapiens
cggaaaagggagtggacaggaggggtacagaaccaggctaatgagacaat

SEQ ID NO: 96 - DNA, 50 bp, Homo sapiens
gctggctttcaggatcactatccagcagcagctccgacttccagattccg

SEQ ID NO: 97 - DNA, 50 bp, Homo sapiens
cgctctctggcaaatgtagaggctatttctgctttttacaagaggtgctg

SEQ ID NO: 98 - DNA, 50 bp, Homo sapiens
cggccctccaaaattgcccccacattggctgccttataaatatgtctgtg

SEQ ID NO: 99 - DNA, 50 bp, Homo sapiens
cgggttcagtcattgaaagccttcttgtaattgctgaagggtatttgttt

SEQ ID NO: 100 - DNA, 50 bp, Homo sapiens
cctctttctgctcgccgaaggccgcgatggtgccataggtgagcttttcg

SEQ ID NO: 101 - DNA, 50 bp, Homo sapiens
cgcctcctgagcctgactctgctcttcccgcagctttggccccccggggc

SEQ ID NO: 102 - DNA, 50 bp, Homo sapiens
cgggcacgatgtcccaggaggacagagtttgcattgatgaaaacccttcc

SEQ ID NO: 103 - DNA, 50 bp, Homo sapiens
cgctgggtctgctcccattggctcaggtcatctgagcagctgtgctctgt

SEQ ID NO: 104 - DNA, 50 bp, Homo sapiens
ggtgctctggaccggcagccatgggaatgtcctagtcggcagcagtgtcg

SEQ ID NO: 105 - DNA, 50 bp, Homo sapiens
ctcacgtacagtctcctccctgtacacgaaggagactctgctctaacacg

SEQ ID NO: 106 - DNA, 50 bp, Homo sapiens
cgctgggatcgtggcttatggcgcagagacttccccatgaccaatcattc

SEQ ID NO: 107 - DNA, 50 bp, Homo sapiens
cgggcaccctgaggttgcccccattctttgaacagctatggacggggacc

SEQ ID NO: 108 - DNA, 50 bp, Homo sapiens
cgggcttcccggcagcaggttactctttaacgctcgactgcccacctcca

SEQ ID NO: 109 - DNA, 50 bp, Homo sapiens
cgccctgattggatagtagtgcaggcaccgcgccctcaggccttgcgtgt

SEQ ID NO: 110 - DNA, 50 bp, Homo sapiens
cgcaactgcagtttagcctggtgagttgcaattctggctgcacatgaaaa

SEQ ID NO: 111 - DNA, 50 bp, Homo sapiens
agttttacaagccctcacataaatctacacagctaacatgcacaagtccg

SEQ ID NO: 112 - DNA, 50 bp, Homo sapiens
cgccttgcgcgctcggcatgacgtcactcccaccaggcacctcgccttgt

SEQ ID NO: 113 - DNA, 50 bp, Homo sapiens
aggcgatccttgcgcttgggcagacagcacgtcacggcttttatctgccg

SEQ ID NO: 114 - DNA, 50 bp, Homo sapiens
agtcagacgtcaggacctgctgtggggatggacccacagctcatcccccg

SEQ ID NO: 115 - DNA, 50 bp, Homo sapiens
cccagtactttgggacgccaaggtgggtgggtcacaaggtcaggagatcg

SEQ ID NO: 116 - DNA, 50 bp, Homo sapiens
taccccagctaggccccttccccgcagaggatgtgtttctgttgtcctcg

SEQ ID NO: 117 - DNA, 50 bp, Homo sapiens
gaggtgggcgaggcagggcccacagacattggtgcaggctcagccgtgcg

SEQ ID NO: 118 - DNA, 50 bp, Homo sapiens
cgactggccacacaatggccaggtagcggtcaacactcatgcaagtgagc

SEQ ID NO: 119 - DNA, 50 bp, Homo sapiens
cttcccctcagccttggtttccatatctggaagatgggttaccaatagcg

SEQ ID NO: 120 - DNA, 50 bp, Homo sapiens
atgtcacttgcacaagagccagtcatgccacagggctagccttaatttcg

SEQ ID NO: 121 - DNA, 50 bp, Homo sapiens
aaataacttgtcctttacttaccctgcacatcaaatcttctcgccctgcg

SEQ ID NO: 122 - DNA, 50 bp, Homo sapiens
atttttattttattcctgccattgtttctccttcgagtcaatatcttccg

SEQ ID NO: 123 - DNA, 50 bp, Homo sapiens
gggcgccagccggcgaggagcgacgggagcctggggtgggtggcgaggcg

SEQ ID NO: 124 - DNA, 50 bp, Homo sapiens
cggctgtggtttcctgtgcgtcccaggtgagatcttgctctttacagggt

SEQ ID NO: 125 - DNA, 50 bp, Homo sapiens
aggacgacaaatggcaagatgtgagttgtggccaaggcgcgcgggcagcg

SEQ ID NO: 126 - DNA, 50 bp, Homo sapiens
cgggcttagtaagcccctggagaaaggaatcaaagatgtttctgaggcct

SEQ ID NO: 127 - DNA, 50 bp, Homo sapiens
cgctggccaccctcctaaaggatcactgtggtgccaggcaggaatgagct

SEQ ID NO: 128 - DNA, 50 bp, Homo sapiens
cggtgtgcaaacctgcaatgaattgcccagtgccttcttgtttgtaacgt

SEQ ID NO: 129 - DNA, 50 bp, Homo sapiens
attatagagaatattaagatgcttttggatcctgagcttcccaggaagcg

SEQ ID NO: 130 - DNA, 50 bp, Homo sapiens
cggctgggtctcatctgacacgcagccttccagcctctcattgcccgagg

SEQ ID NO: 131 - DNA, 50 bp, Homo sapiens
agggaagttgggagtattgtgctcccctgagagccgttgccacggttacg

SEQ ID NO: 132 - DNA, 50 bp, Homo sapiens
ccagcagcagcggcagcaaggtttacaatcctaaaccatgcaggcttccg

SEQ ID NO: 133 - DNA, 50 bp, Homo sapiens
tagccatttggcctcggcatcacggtgcgggagcgtggggcgcagactcg

SEQ ID NO: 134 - DNA, 50 bp, Homo sapiens
caagcaagactctccacccacaaactgcatattctttaaagtcactgtcg

SEQ ID NO: 135 - DNA, 50 bp, Homo sapiens
cgcttaaggaccttatagctagcaaatggcagagacaagcttggggcaga

SEQ ID NO: 136 - DNA, 50 bp, Homo sapiens
agatgttatcagctcagcgagactttccatgatctccctaaaatgaatcg

SEQ ID NO: 137 - DNA, 50 bp, Homo sapiens
cgcccagaactgggacttcccaggttctcatagtgattgtagatatcaat

SEQ ID NO: 138 - DNA, 50 bp, Homo sapiens
gctagtgagccgcgcgctgggccggcagcagggggttattttagtgcgcg

SEQ ID NO: 139 - DNA, 50 bp, Homo sapiens
ggctggaggcggctgggggcccggccagtgcgccaggagccgcaggaacg

SEQ ID NO: 140 - DNA, 50 bp, Homo sapiens
ggcaggcaggcggcaggcagagcgcgctctccgggcagtctgaaggaccg

SEQ ID NO: 141 - DNA, 50 bp, Homo sapiens
cgctccgccggtgctcgctctatttgaaaacgctgactgttggtccccca

SEQ ID NO: 142 - DNA, 50 bp, Homo sapiens
acagaaccccagaaaaactgtcccacaacccccagtgaatgaccaaatcg

SEQ ID NO: 143 - DNA, 50 bp, Homo sapiens
cggaagctgcaccctaaattccccgggacctgtggcaggccttcctggtg

SEQ ID NO: 144 - DNA, 50 bp, Homo sapiens
agccacgaagaaaacagttcaactcagaccaaaagataaagctgatctcg

SEQ ID NO: 145 - DNA, 50 bp, Homo sapiens
gcctggtccccgaaagcgctcagtcagaatccgagagcactgtggcggcg

SEQ ID NO: 146 - DNA, 50 bp, Homo sapiens
cgcctctcacagactgcttccccagcagggtgcagcttcttacagactgg

SEQ ID NO: 147 - DNA, 50 bp, Homo sapiens
tgattcagtccagtgattgggtttgtggctccaggcctcgcccacagacg

SEQ ID NO: 148 - DNA, 50 bp, Homo sapiens
cgtctcgccttgcgagcaagctcggaatccagttcctcaggaacccctcc

SEQ ID NO: 149 - DNA, 50 bp, Homo sapiens
cagcaaagaaatgactatagttggaacacaggacttttgcctcctgcccg

SEQ ID NO: 150 - DNA, 50 bp, Homo sapiens
cccatccatgacttcttatgtgtgctgtcggcagctgaccagcggccacg

SEQ ID NO: 151 - DNA, 50 bp, Homo sapiens
aggcagcagcccagtggcctcttgctgtggagcgcgggggcagcctcccg

SEQ ID NO: 152 - DNA, 50 bp, Homo sapiens
cgggtgttgtgtctctgcctatcttcacacatgcacccttgtgaacttgg

SEQ ID NO: 153 - DNA, 50 bp, Homo sapiens
cggactcattgccatgcatgcctagacattaatatgtgttcatggagggc

SEQ ID NO: 154 - DNA, 50 bp, Homo sapiens
tgtgctcagattcacaaagtgaaagtgcaaaaccccgtgttagctcatcg

SEQ ID NO: 155 - DNA, 50 bp, Homo sapiens
cgggctatagcgagaccccccatagtgagatctgctgcgggacctagagt

SEQ ID NO: 156 - DNA, 50 bp, Homo sapiens
cggtggcctgttgaggcccaactcatgcctctggcaccctttcaagaggc

SEQ ID NO: 157 - DNA, 50 bp, Homo sapiens
gcaaggtgaacccaccttgatcccggggctgcagagccagtgcgcctgcg

SEQ ID NO: 158 - DNA, 50 bp, Homo sapiens
cggttggcaagagcttggctagagagactgatgtagatggcagcttctta

SEQ ID NO: 159 - DNA, 50 bp, Homo sapiens
cgagaggcatttcagcagaattttgaaggtggagtgaaggaagtcactat

SEQ ID NO: 160 - DNA, 50 bp, Homo sapiens
aaacactctcccggctcagaaacggtgcaggtgcatttacatgtcaatcg

SEQ ID NO: 161 - DNA, 50 bp, Homo sapiens
cgcgggctctatctgcagcatccaccccctcagcagacgctggcataagc

SEQ ID NO: 162 - DNA, 50 bp, Homo sapiens
ggggccgcagtgtccttggctcaggcctcctacgcagggaagcagggtcg

SEQ ID NO: 163 - DNA, 50 bp, Homo sapiens
cgggaaagtatcacttgtgactgtttgcactaggtgcaaaagacagatag

SEQ ID NO: 164 - DNA, 50 bp, Homo sapiens
tctgtagagaagtcgaccgagaagtgagatgcggtggcgacctcggagcg

SEQ ID NO: 165 - DNA, 50 bp, Homo sapiens
cgctgcccatgcccagaccaaaaatggggtgtctttttagtctaaaagga

SEQ ID NO: 166 - DNA, 50 bp, Homo sapiens
cggccagacccgtcactcagatccccgcaccaggccagtgaagaggagcc

SEQ ID NO: 167 - DNA, 50 bp, Homo sapiens
ccagcccttctggcacagatgctgtgcatgtgaggtgcttctcagaagcg

SEQ ID NO: 168 - DNA, 50 bp, Homo sapiens
aggagatgagctatgtcttccaacctctccttttggaataaaacctttcg

SEQ ID NO: 169 - DNA, 50 bp, Homo sapiens
cgacgacaaagaagattttgatgaagttcaaattagagtcagcgtgctca

SEQ ID NO: 170 - DNA, 50 bp, Homo sapiens
gtaaagtgacacccatcccactcatcccattgctgccaatgacttcaacg

SEQ ID NO: 171 - DNA, 50 bp, Homo sapiens
caccttccactttaaagaacaccaaggtcggctgggtgtggtggctcacg

SEQ ID NO: 172 - DNA, 50 bp, Homo sapiens
cgagcccaggaaataagtgcgggtgaccgaattcaatcctgcatccaaca

SEQ ID NO: 173 - DNA, 50 bp, Homo sapiens
cggccccacttagcctgaaacggggccccatgcagggtagaggcctgcca

SEQ ID NO: 174 - DNA, 50 bp, Homo sapiens
cgcacaccgagtggcacgacctgcagaggttaccgccaggtttccatcct

SEQ ID NO: 175 - DNA, 50 bp, Homo sapiens
tggggtgagccactttcattttcccagcggggccaggcagtctttgctcg

SEQ ID NO: 176 - DNA, 50 bp, Homo sapiens
cgcaggtctgagagacatcacagcatcacagcgtttagtagtcttaaatg

SEQ ID NO: 177 - DNA, 50 bp, Homo sapiens
cgactaccactgctggtgcaaggaccaatcagcgacctattgaagtgcct

SEQ ID NO: 178 - DNA, 50 bp, Homo sapiens
cgggatggtgtgacaggcaagccaaagttgtatctgaaaactctgcaaca

SEQ ID NO: 179 - DNA, 50 bp, Homo sapiens
ggtccgctggggcagagtgcggagtgaaggggtgcactgggcactcagcg

SEQ ID NO: 180 - DNA, 50 bp, Homo sapiens
ctttaagatgtctgacagtgccctaagggcacgtgctccacaaacaaacg

SEQ ID NO: 181 - DNA, 50 bp, Homo sapiens
ctcaaagaaaataagccaggaccaggtgacccagtgggatccgcgaagcg

SEQ ID NO: 182 - DNA, 50 bp, Homo sapiens
tgcggccactgcaaagcgatgtaaatgtcccagagtggggcagctggtcg

SEQ ID NO: 183 - DNA, 50 bp, Homo sapiens
cgtgccacctggccaacctcgaaaggaggccctgctgggttcttcatctt

SEQ ID NO: 184 - DNA, 50 bp, Homo sapiens
cggcggacccagctgaccaaaggaactacagaagaggacgaagaaagcga

SEQ ID NO: 185 - DNA, 50 bp, Homo sapiens
tcgctttccagccttttgtttctggatcctcaaaactcagaacgtggccg

SEQ ID NO: 186 - DNA, 50 bp, Homo sapiens
tggagcaaatataggtctagacacgtagggcctgtgaggttttcctgacg

SEQ ID NO: 187 - DNA, 50 bp, Homo sapiens
gcgtgtgctcagcgtgtggttaccgtgtgcacagcacgagcttgaactcg

SEQ ID NO: 188 - DNA, 50 bp, Homo sapiens
cgtggccactcttcagcatctctgtcggaagaccgtcaacggccacctgg

SEQ ID NO: 189 - DNA, 50 bp, Homo sapiens
cgggaatggtgactcagccttccaggaacctgcgtggcgtctgttttttt

SEQ ID NO: 190 - DNA, 50 bp, Homo sapiens
cgggcgcagccccaggatgcaacagctctcatacaattggccaggaaggc

SEQ ID NO: 191 - DNA, 50 bp, Homo sapiens
cgggtttcccaagtgctggacgcgcaacaggtttccataaacccaaagtt

SEQ ID NO: 192 - DNA, 50 bp, Homo sapiens
cggcgagtgagtgaaaaattacattttcacttgggttctgaacattcagt

SEQ ID NO: 193 - DNA, 50 bp, Homo sapiens
cggggaaactctgaattggtggttgcttagaaaacacatagaagtgtgta

SEQ ID NO: 194 - DNA, 50 bp, Homo sapiens
tcagggttgaaaacgcaacagccaaaattaactcagtggatggctcaacg

SEQ ID NO: 195 - DNA, 50 bp, Homo sapiens
cgccggtggccgacggcttctgaggaattatcttttacttggcgccacac

SEQ ID NO: 196 - DNA, 50 bp, Homo sapiens
cgagattaaagattcagaaagtgagtaaagttaacactgagcccttgggc

SEQ ID NO: 197 - DNA, 50 bp, Homo sapiens
agttggtgagccagggaagtcttccctcgccctgagggtgcggggaagcg

SEQ ID NO: 198 - DNA, 50 bp, Homo sapiens
cggggccaaagaggagcgcaggtttaaaaagcaagtgtattagcaagttt

SEQ ID NO: 199 - DNA, 50 bp, Homo sapiens
cgcccacgcggacccctctccgtgtgcttgtctgtacttccctgatgggg

SEQ ID NO: 200 - DNA, 50 bp, Homo sapiens
cggccggagggccctgaaccctaggccaagactcatccacaacctagggg

SEQ ID NO: 201 - DNA, 50 bp, Homo sapiens
cgggagatcctcccgcggccggagggccctgaaccctaggccaagactca

SEQ ID NO: 202 - DNA, 50 bp, Homo sapiens
cgtgagcgggatcctgagtctgagttgccgcttaacccggcattttataa

SEQ ID NO: 203 - DNA, 50 bp, Homo sapiens
cggaggcaagcaagctccatgtggtggggacagcgcattgcgacctccac

SEQ ID NO: 204 - DNA, 50 bp, Homo sapiens
ccatgctataagtgaggtaaataaatatgctgagcaccatcgcacttacg

SEQ ID NO: 205 - DNA, 50 bp, Homo sapiens
cgcggcattcagcagaactcatgatgaaggaaacagttccatggcagggt

SEQ ID NO: 206 - DNA, 50 bp, Homo sapiens
cgacaaaatctgaccaggctagatctgaatctgttaatttctgagacggt

SEQ ID NO: 207 - DNA, 50 bp, Homo sapiens
cgcagaggagaatgtcagatgctcagctcggtcccctccgcctgacgctc

SEQ ID NO: 208 - DNA, 50 bp, Homo sapiens
cgcccgattcagacagctggactcagagggattctgctccacagagaaac

SEQ ID NO: 209 - DNA, 50 bp, Homo sapiens
cgtatgtgtttgagatagcagttgtttactatcacttgaaaattctgaat

SEQ ID NO: 210 - DNA, 50 bp, Homo sapiens
tcatgaactggagcctgaagtggctctgaggcctcccctggaaaggaacg

SEQ ID NO: 211 - DNA, 50 bp, Homo sapiens
cggtggattcctctcgggacacatctgccacccgctggactggcaaaaca

SEQ ID NO: 212 - DNA, 50 bp, Homo sapiens
cgaccatttgtatgtgtatctatgtcagaaagaatctttattaaaatatt

SEQ ID NO: 213 - DNA, 50 bp, Homo sapiens
taccatgtaatataccactaaacacacactatgtaatacactactaaacg

SEQ ID NO: 214 - DNA, 50 bp, Homo sapiens
ttgtctcagattacaggaaccaaatgcatgtctggccttgtgctgcttcg

SEQ ID NO: 215 - DNA, 50 bp, Homo sapiens
cgagcccgcccagcctctgaacctccgtgtcttcatctgtaaattgaggg

SEQ ID NO: 216 - DNA, 50 bp, Homo sapiens
gtgctctcagtccaattcacactgaatgaatgaatcagtcccagccatcg

SEQ ID NO: 217 - DNA, 50 bp, Homo sapiens
cgctgaggtcccgtttctgtagctgagtagcccggtgacactgccctccg

SEQ ID NO: 218 - DNA, 50 bp, Homo sapiens; identical to SEQ ID NO: 6

SEQ ID NO: 219 - DNA, 50 bp, Homo sapiens
cgccgcagtcccagtcgagccgcgacccttccggctgcccccaccccacc

SEQ ID NO: 220 - DNA, 50 bp, Homo sapiens
tgtgccttgacgggctgtcccaggcgcccctggaattgatgcagtgtccg

SEQ ID NO: 221 - DNA, 50 bp, Homo sapiens
cgcagaagaaagctgctcaagtgctggagtggccaaccccatgccgttcc

SEQ ID NO: 222 - DNA, 50 bp, Homo sapiens
cgcacatcctcagctagcagcatggagctgagttcagaggaggcacttag

SEQ ID NO: 223 - DNA, 50 bp, Homo sapiens
cgggagggaaaggtgttagatggtggttttaactcaccagggtttgaatt

SEQ ID NO: 224 - DNA, 50 bp, Homo sapiens
cggcctgattcgaagactggaatagaggatttctagaattctgtgactcc

SEQ ID NO: 225 - DNA, 50 bp, Homo sapiens
catgtcccagctcagctggtcctgagaagctgcctggtagacagtcaccg

SEQ ID NO: 226 - DNA, 50 bp, Homo sapiens
tagaaccaactggatactgcacccctcagtattggggcgtcacagcaccg

SEQ ID NO: 227 - DNA, 50 bp, Homo sapiens; identical to SEQ ID NO: 176

SEQ ID NO: 228 - DNA, 50 bp, Homo sapiens
caagtcctttctggttcccgtggtttttcaggtactgcggttcttattcg

SEQ ID NO: 229 - DNA, 50 bp, Homo sapiens
ctccctacgtgggggacgtgcaggatgatgcggggtcgggggggatttcg

SEQ ID NO: 230 - DNA, 50 bp, Homo sapiens
tccgcaaaaagcaggatccattcactttagagaagtgccctcaacaggcg

SEQ ID NO: 231 - DNA, 50 bp, Homo sapiens
tgtggtctccccagaccaccaggtgcttcacacacgcacaggggcactcg

SEQ ID NO: 232 - DNA, 50 bp, Homo sapiens
tgcagcctcgtaagcctcatggaagagcttggtttgtatcctttggaacg

SEQ ID NO: 233 - DNA, 50 bp, Homo sapiens
cagtgctgagccggatccagaaaattgaacaggtcctgaaggagcagccg

SEQ ID NO: 234 - DNA, 50 bp, Homo sapiens
cgtccccgaaatgaataatgcaggcaggagccaagatttctgcattagcg

SEQ ID NO: 235 - DNA, 50 bp, Homo sapiens
cggtgtggaggctttttttgtcagaagctctggggtttggctcttctctg

SEQ ID NO: 236 - DNA, 50 bp, Homo sapiens
cctctttgctgatctggactcagcctggtattcttgtcacaaggtcatcg

SEQ ID NO: 237 - DNA, 50 bp, Homo sapiens
tttttaaccagtttgaacattttactacttcctaacatcagaagcacccg

SEQ ID NO: 238 - DNA, 50 bp, Homo sapiens
gtgtggcaaggctgagctagttcgtctgccaggtaccagagcaagcctcg

SEQ ID NO: 239 - DNA, 50 bp, Homo sapiens
cactatgtttgctgcttgctattcacttatggtacatacacagtcagtcg

SEQ ID NO: 240 - DNA, 50 bp, Homo sapiens
gggacggtggtagtgcttctcaacattggcactggctccattgtcattcg

SEQ ID NO: 241 - DNA, 50 bp, Homo sapiens
tggggagccagctgacttaacaggcctggattacattcttgcttccaacg

SEQ ID NO: 242 - DNA, 50 bp, Homo sapiens
tgccatttaatctaacgccaccttctacggaccagagcaggtgctctgcg

SEQ ID NO: 243 - DNA, 50 bp, Homo sapiens
cggttaaattcgtgaggctgtttgctgtgtacacaatgctaagcagaaaa

SEQ ID NO: 244 - DNA, 50 bp, Homo sapiens; identical to SEQ ID NO: 182

SEQ ID NO: 245 - DNA, 50 bp, Homo sapiens
tctggtcctggcctgggggggtcgtggtctcgctggtgcagcctcctccg

SEQ ID NO: 246 - DNA, 50 bp, Homo sapiens
cgccaccatcgagtgtgagcagccccagcccgacctctacaagtaagcgg

SEQ ID NO: 247 - DNA, 50 bp, Homo sapiens
cgctgtgaaacctttgcctttgggtgtcatggtggaagcaaatcttagaa

SEQ ID NO: 248 - DNA, 50 bp, Homo sapiens
cgccagggcaaacattccttgggcgcctcgggcttttccctagggaagca

SEQ ID NO: 249 - DNA, 50 bp, Homo sapiens; identical to SEQ ID NO: 185

SEQ ID NO: 250 - DNA, 50 bp, Homo sapiens
cggagagacagccgctgtggttaggggtgtgcatccttctaccatgccca

SEQ ID NO: 251 - DNA, 50 bp, Homo sapiens
cgtggatctagccacagaaaggcaacagcgcttcaaagaggctctccgta

SEQ ID NO: 252 - DNA, 50 bp, Homo sapiens
cgcttttgcaaaacaggccgcacctagcccagattctggagctgattcag

SEQ ID NO: 253 - DNA, 50 bp, Homo sapiens
cgactctgagttctgacagggaaatacaatgagttttatgtggacagagt

SEQ ID NO: 254 - DNA, 50 bp, Homo sapiens
ctctctcccagacctcaggtaaaattaatgttctaggaacgtatgccacg

SEQ ID NO: 255 - DNA, 50 bp, Homo sapiens
tggggtggccgtctgctccgtctttggtggtgagaacccgcaccggtccg

SEQ ID NO: 256 - DNA, 50 bp, Homo sapiens
cggtgtctccgctccttgcccgtggccaggtggtggtgctcccaatgccc

SEQ ID NO: 257 - DNA, 50 bp, Homo sapiens
cgggctttaaggtggcccttgcagatcttgcagacattttcgtgggctcc

SEQ ID NO: 258 - DNA, 50 bp, Homo sapiens
agactccctctgaacacctgtggaacatgctgacctcccagtgtctttcg

SEQ ID NO: 259 - DNA, 50 bp, Homo sapiens
cgcacatgtgaggccaccattcataccacaccctgggtgggtcttgagtt

SEQ ID NO: 260 - DNA, 50 bp, Homo sapiens
tctgctcattaacaccctgttaataggaaccccagaaacctgagcttccg

SEQ ID NO: 261 - DNA, 50 bp, Homo sapiens
cggccttgcacaccatcttaagtgtgacgccacactgcccttcacagcct

SEQ ID NO: 262 - DNA, 50 bp, Homo sapiens; identical to SEQ ID NO: 188

SEQ ID NO: 263 - DNA, 50 bp, Homo sapiens
cgcgcctggtgcagccctcacctcaccaggtgttgatcatcttagtggtt

SEQ ID NO: 264 - DNA, 50 bp, Homo sapiens
cgcacttaatatgattattttttgatgccaggtccaccaagtgaagattg

SEQ ID NO: 265 - DNA, 50 bp, Homo sapiens
cgtgtaaaggtcagaggtccattcaccaatgcaatgatcctcactgcccc

SEQ ID NO: 266 - DNA, 50 bp, Homo sapiens; identical to SEQ ID NO: 189

SEQ ID NO: 267 - DNA, 50 bp, Homo sapiens
tattgcagtatcctaaagcgtgctgtatctctctgtccggcttttgcacg

SEQ ID NO: 268 - DNA, 50 bp, Homo sapiens
cggtcttgtaacaattggatggatgcctttgaagagcccctgtccctatt

SEQ ID NO: 269 - DNA, 50 bp, Homo sapiens
tctcctcccctgcactggctctgggtgcttatctctgcagaagcttctcg

SEQ ID NO: 270 - DNA, 50 bp, Homo sapiens
cggggtctagggaagagagatttcctaacctagactacaggcatcaggag

SEQ ID NO: 271 - DNA, 50 bp, Homo sapiens
tgattcctccccctttgaaagagcaggcagcatttttccaaggcaacccg

SEQ ID NO: 272 - DNA, 50 bp, Homo sapiens
cgctggtctcgggggggaacccaacagactcacatttcatgtgaaaggaa

SEQ ID NO: 273 - DNA, 50 bp, Homo sapiens
aaagatgtcattacacaaatacacaaatactagcatgcagacacacaacg

SEQ ID NO: 274 - DNA, 50 bp, Homo sapiens
gatgtatctcccacccaggagtgtttcttggccaggtgtggtggctcacg

SEQ ID NO: 275 - DNA, 50 bp, Homo sapiens
cgacaactctgtagtgatttagaagagaattgcaagacattaacacagag

SEQ ID NO: 276 - DNA, 50 bp, Homo sapiens; identical to SEQ ID NO: 193

SEQ ID NO: 277 - DNA, 50 bp, Homo sapiens
gtttcagcacctgggtcagcgcttcccagggtcagcaccagggatagacg

SEQ ID NO: 278 - DNA, 50 bp, Homo sapiens
cgcagctgtcgtctttgtacccggctttgcgcactccattgtggacgcga

SEQ ID NO: 279 - DNA, 50 bp, Homo sapiens; identical to SEQ ID NO: 124

SEQ ID NO: 280 - DNA, 50 bp, Homo sapiens
gcacctttgtgaggtgtttgtggggttgggggagcttcaggcgctactcg

SEQ ID NO: 281 - DNA, 50 bp, Homo sapiens
cggtacttccctgatggggcccacgcggacccctctccagtgtgcttgtc

SEQ ID NO: 282 - DNA, 50 bp, Homo sapiens
atcttcccagtacagagcttagcatacattgaataactggcatctgctcg

SEQ ID NO: 283 - DNA, 50 bp, Homo sapiens
actctgtcagatatcctcgatatttggggatagtagttcaaaaacagccg

SEQ ID NO: 284 - DNA, 50 bp, Homo sapiens
agctgtttccctcaggcggcctgttccacgccaggattagttttgcttcg

SEQ ID NO: 285 - DNA, 50 bp, Homo sapiens
cggtttgcaggttcaaagatgtctaaaagagaatggccagaatgtatata

SEQ ID NO: 286 - DNA, 50 bp, Homo sapiens
atccctcatctggactttgagtgattgtgttgctggcatggaccctttcg

SEQ ID NO: 287 - DNA, 50 bp, Homo sapiens
cagagcccacttagtgcgcgctagctgggcagggataggggtcctattcg

SEQ ID NO: 288 - DNA, 50 bp, Homo sapiens
acagtatttttgtcactccaagtatcccttatcttgcccttttatggtcg

SEQ ID NO: 289 - DNA, 50 bp, Homo sapiens
ctgaaaggcgcattgtcagcctggggaggcgacgcggcgcgaggacagcg

SEQ ID NO: 290 - DNA, 50 bp, Homo sapiens
cggagggcttattctatgtaaatagttgaaaggaactggataagactgta

SEQ ID NO: 291 - DNA, 50 bp, Homo sapiens; identical to SEQ ID NO: 205

SEQ ID NO: 292 - DNA, 50 bp, Homo sapiens
cgcccagctggaggctgagatgtcaggatttgtcttgcaaagttacttca

SEQ ID NO: 293 - DNA, 50 bp, Homo sapiens
cgcaaaacttaaggctatagaagatggggagagtatcttttgatgcagac

SEQ ID NO: 294 - DNA, 50 bp, Homo sapiens; identical to SEQ ID NO: 207

SEQ ID NO: 295 - DNA, 50 bp, Homo sapiens; identical to SEQ ID NO: 208

SEQ ID NO: 296 - DNA, 50 bp, Homo sapiens
cgctgcactcagccacgttacgcggagttcatctggggaaggagacaaat

SEQ ID NO: 297 - DNA, 50 bp, Homo sapiens
gaagggtcacacatgtcccagaatcccccaggagtgatgcaaatggagcg

SEQ ID NO: 298 - DNA, 50 bp, Homo sapiens
aaaccctaaacactgaagtctcctctggtcaggtgacccctatcagtccg

SEQ ID NO: 299 - DNA, 50 bp, Homo sapiens
gccaggagtcctcggtcctgggagggtttaaaagccagggggccgtctcg

SEQ ID NO: 300 - DNA, 50 bp, Homo sapiens
gaccctgggcttggggggatttttttggcctggagggctcctcttctccg

SEQ ID NO: 301 - DNA, 50 bp, Homo sapiens
ggccagacacccaggacccaaataacctaataatggctcatttgcctccg

SEQ ID NO: 302 - DNA, 50 bp, Homo sapiens
cggcattggtcctttattgaacatcctcccaaagctggggctagggttca

SEQ ID NO: 303 - DNA, 50 bp, Homo sapiens
ccagatgttttcactcgattttgcaaatctgctccaggtctaagacatcg

SEQ ID NO: 304 - DNA, 50 bp, Homo sapiens
cgggtcttcactctggttggctgccagatcctccaggggcggggtctcac

SEQ ID NO: 305 - DNA, 50 bp, Homo sapiens
tacagaacccctgaaacattcctgccaaatacagtcgcacgaatttgtcg

SEQ ID NO: 306 - DNA, 50 bp, Homo sapiens; identical to SEQ ID NO: 173

SEQ ID NO: 307 - DNA, 50 bp, Homo sapiens
cgcacagcaactggggtgtcctgaccagtgagctagagttccaccttact

SEQ ID NO: 308 - DNA, 50 bp, Homo sapiens
ttataatccaaaaatatttattaaccatctgctctgtgacaagcactgcg

SEQ ID NO: 309 - DNA, 50 bp, Homo sapiens
ctttggctcgagctccaggtgcagatttacgttcattttcttttgttccg

SEQ ID NO: 310 - DNA, 50 bp, Homo sapiens
aaaaacttttctgagccggagcctccagcgcgctgtgtattcgttttacg

SEQ ID NO: 311 - DNA, 50 bp, Homo sapiens; identical to SEQ ID NO: 221

SEQ ID NO: 312 - DNA, 50 bp, Homo sapiens
cgcagattccccatttgtgagcagagttaagctgaaggagcgtgggcatg

SEQ ID NO: 313 - DNA, 50 bp, Homo sapiens
cggccccagaaggcaaggcgattgttaggaggaattaaacaggctagtgc

SEQ ID NO: 314 - DNA, 50 bp, Homo sapiens
cgcccggcgaccactggtggttctatgctgctggggtgaaaagtctgaag

SEQ ID NO: 315 - DNA, 50 bp, Homo sapiens
aggacactggccagcctccagttggtttctgaagctagcagtcttagtcg

SEQ ID NO: 316 - DNA, 50 bp, Homo sapiens
cgccctgccctgggattctcagaccttgaaagccacaagtcttgaaagtc

SEQ ID NO: 317 - DNA, 50 bp, Homo sapiens; identical to SEQ ID NO: 176

SEQ ID NO: 318 - DNA, 50 bp, Homo sapiens; identical to SEQ ID NO: 229

SEQ ID NO: 319 - DNA, 50 bp, Homo sapiens
ctgaattctggtacctgttaatgacagcttctgagaggtttcttttatcg

SEQ ID NO: 320 - DNA, 50 bp, Homo sapiens
taaccttgaacaaagatcgtcgacgggcggccctcactggaaacctttcg

SEQ ID NO: 321 - DNA, 50 bp, Homo sapiens; identical to SEQ ID NO: 234

SEQ ID NO: 322 - DNA, 50 bp, Homo sapiens
cgagttgtaagtcaacctgctgggttgtgctgaagagaaattggagactg

SEQ ID NO: 323 - DNA, 50 bp, Homo sapiens
ttagggcctggagatgggcagacccaggctcacatcctagctctgacacg

SEQ ID NO: 324 - DNA, 50 bp, Homo sapiens
cggctctaagcggggcaagagctgcttttaatttgagacgtacacagttt

SEQ ID NO: 325 - DNA, 50 bp, Homo sapiens; identical to SEQ ID NO: 237

SEQ ID NO: 326 - DNA, 50 bp, Homo sapiens
acacataccccactaaagaagattcacaaggttgggtgcagtggttcacg

SEQ ID NO: 327 - DNA, 50 bp, Homo sapiens
actatgtacctggaaatagcaggggctcagggtttgatcctatgagaccg

SEQ ID NO: 328 - DNA, 50 bp, Homo sapiens
cggctacgagcacagagcatcatcatcatcagcctgccagccggccccgc

SEQ ID NO: 329 - DNA, 50 bp, Homo sapiens; identical to SEQ ID NO: 251

SEQ ID NO: 330 - DNA, 50 bp, Homo sapiens
cctctggacagtacttttgagacacacttatttctaccacgcaccttgcg

SEQ ID NO: 331 - DNA, 50 bp, Homo sapiens
cgagaagttcaagttcaagctgcagaacaccagtgtgcagaaggagcact

SEQ ID NO: 332 - DNA, 50 bp, Homo sapiens
cgcgcaggaaaagggaaacaaacagcagcttcgcagcctccctgggcctg

SEQ ID NO: 333 - DNA, 50 bp, Homo sapiens
ctatggtcaactgagtcagggctggatttctcacccaccctggccaatcg

SEQ ID NO: 334 - DNA, 50 bp, Homo sapiens
cgctcctattcaccgaacccctggctggctgacccgggaaaaacagtcta

SEQ ID NO: 335 - DNA, 50 bp, Homo sapiens
tccaccaggtctcttatcaatggacagtacaaacagtactaccacgaacg

SEQ ID NO: 336 - DNA, 50 bp, Homo sapiens
cgcgtgtttctctgcgctgtggtcgtcatggaccggaagcgtgtgcagcg

SEQ ID NO: 337 - DNA, 50 bp, Homo sapiens
ttttcttctttggcttttccatcactgctggctacaagtgtttgcaaccg

SEQ ID NO: 338 - DNA, 50 bp, Homo sapiens
ggggttgccggcaccttctctttctccccaggtcctttcatctgattccg

SEQ ID NO: 339 - DNA, 50 bp, Homo sapiens; identical to SEQ ID NO: 188

SEQ ID NO: 340 - DNA, 50 bp, Homo sapiens
cgcacggcctccagcagcaagctgatgctgtcctacaagaagccaaaagg

SEQ ID NO: 341 - DNA, 50 bp, Homo sapiens; identical to SEQ ID NO: 265

SEQ ID NO: 342 - DNA, 50 bp, Homo sapiens
gtcctaaagcaccaggatagatgacgagcagggccaagtccacacaagcg

SEQ ID NO: 343 - DNA, 50 bp, Homo sapiens
tttaagctatcaatgtggatgtgctggtgctgagacccacctccaacacg

SEQ ID NO: 344 - DNA, 50 bp, Homo sapiens; identical to SEQ ID NO: 189

SEQ ID NO: 345 - DNA, 50 bp, Homo sapiens
ctcctccgagtagccggcgccgtggatgatgcgcatctgcttgatgaacg

SEQ ID NO: 346 - DNA, 50 bp, Homo sapiens
actggaccctcggctcttccttggacttcttgtgtgttctgtgagcttcg

SEQ ID NO: 347 - DNA, 50 bp, Homo sapiens
tggggctttaaaaaccacagcccttgggcaggagggaccttcgatcctcg

SEQ ID NO: 348 - DNA, 50 bp, Homo sapiens
cgctccctcttaggtcacctgccatttcagacagggaagagaacagtgaa

SEQ ID NO: 349 - DNA, 50 bp, Homo sapiens
agcagctccaccggggatgcggctcgtcagggggtgtacgagaacttccg

SEQ ID NO: 350 - DNA, 50 bp, Homo sapiens; identical to SEQ ID NO: 274

SEQ ID NO: 351 - DNA, 50 bp, Homo sapiens
cgccacagagggcttccccaggtccaggccgggccagccttgacctctaa

SEQ ID NO: 352 - DNA, 50 bp, Homo sapiens
cgaacctgatgtggagacaaagtatccttcatggactttgaatttgatat

SEQ ID NO: 353 - DNA, 50 bp, Homo sapiens
aagggtagctgctgccactgctacattctacagaaagctcaatgagtccg

SEQ ID NO: 354 - DNA, 50 bp, Homo sapiens
cggctccctcacacccactgagagcatcatgtccctgggcacgcactccc

SEQ ID NO: 355 - DNA, 50 bp, Homo sapiens; identical to SEQ ID NO: 193

SEQ ID NO: 356 - DNA, 50 bp, Homo sapiens
cgctgcttcaactggagttaaccaagtgaacacagagctttacaaagaac

SEQ ID NO: 357 - DNA, 50 bp, Homo sapiens
ctcggtctcgtgtgtctgtgtgtgccagtcccttgtgctgacacaggacg

SEQ ID NO: 358 - DNA, 50 bp, Homo sapiens
tatgcagttgtaattctgacagtattgccaaattgttcacagtaaagacg

SEQ ID NO: 359 - DNA, 50 bp, Homo sapiens
cggcagagaggcctgagataaggtttttgcacatggctggtaagactgga

SEQ ID NO: 360 - DNA, 50 bp, Homo sapiens
cggttgtcagcaccatatttctaaaatgcaaatctggcaagtcattttct

SEQ ID NO: 361 - DNA, 50 bp, Homo sapiens
cgcggctgtaccacatagagaaagatatgcactagttcaaagagaatgcc

SEQ ID NO: 362 - DNA, 50 bp, Homo sapiens; identical to SEQ ID NO: 196

SEQ ID NO: 363 - DNA, 50 bp, Homo sapiens
aggccccaaggttcctgacagagctgctgttgggtgttggtgtaaagccg

SEQ ID NO: 364 - DNA, 50 bp, Homo sapiens
aaaaagactgcagctcccatcttaattgctctctcatgcttgtgtgtgcg

SEQ ID NO: 365 - DNA, 50 bp, Homo sapiens
gaattctgctggcgctgcagctgcagaatggtcggcggtggcgggaagcg

SEQ ID NO: 366 - DNA, 50 bp, Homo sapiens
agcttcagacacagtcaacgtgctgccaacgtggggagggccggaggacg

SEQ ID NO: 367 - DNA, 50 bp, Homo sapiens
cggagatgaaattaatgtgaaccactgaggcaaaggcatgaggccccctc

SEQ ID NO: 368 - DNA, 50 bp, Homo sapiens
cggctgccccctcaccagcaccctccgattccagcgacagcctcttggct

SEQ ID NO: 369 - DNA, 50 bp, Homo sapiens
gtccctggagccaggcgttaatcattgacctgattagcaagaacgctccg

SEQ ID NO: 370 - DNA, 50 bp, Homo sapiens
cgacatgacaagatttaagggaggcacatctcacagacaagcatgaaaac

SEQ ID NO: 371 - DNA, 50 bp, Homo sapiens
ctggcccggccgcccctcagctatttgttcacgtaatgcgattggaaacg

SEQ ID NO: 372 - DNA, 50 bp, Homo sapiens
taaatggacttactttgaggccatgatcaacatttaaatcttgctcttcg

SEQ ID NO: 373 - DNA, 50 bp, Homo sapiens; identical to SEQ ID NO: 287

SEQ ID NO: 374 - DNA, 50 bp, Homo sapiens
cggacacttccggtggaaggactgagcggcgctacacttcaagaattccg

SEQ ID NO: 375 - DNA, 50 bp, Homo sapiens
ttattgttttcctgtcttctacagcagaattggatattcccaaacaatcg

SEQ ID NO: 376 - DNA, 50 bp, Homo sapiens
cggggtctgggttttcttgtcccactgggagtttcaagccccaggtagaa

SEQ ID NO: 377 - DNA, 50 bp, Homo sapiens
tcaagggagggcgatattccagtgctgatcccattttcctcccctcctcg

SEQ ID NO: 378 - DNA, 50 bp, Homo sapiens
tcaggaaaactcatgccattctccattcaacggagggcgacattctagcg

SEQ ID NO: 379 - DNA, 50 bp, Homo sapiens
cgtccagcagacaaagactatggtttaatgaaaatagatgaaccaagcac

SEQ ID NO: 380 - DNA, 50 bp, Homo sapiens
actgatgatttccaggaactaccaaagccacggatcagctgagttacccg

SEQ ID NO: 381 - DNA, 50 bp, Homo sapiens; identical to SEQ ID NO: 289

SEQ ID NO: 382 - DNA, 50 bp, Homo sapiens
aacaacaaaaaacttaaatttcccttgacttttaagttcactcttgttcg

SEQ ID NO: 383 - DNA, 50 bp, Homo sapiens; identical to SEQ ID NO: 207

SEQ ID NO: 384 - DNA, 50 bp, Homo sapiens; identical to SEQ ID NO: 208

SEQ ID NO: 385 - DNA, 50 bp, Homo sapiens
tcccaccccttccattctgttgagctgagacgcgtgttttggtcgtttcg

SEQ ID NO: 386 - DNA, 50 bp, Homo sapiens
cctgatttacacttggctccacccataaagttcccactgattatcacacg

SEQ ID NO: 387 - DNA, 50 bp, Homo sapiens; identical to SEQ ID NO: 299

SEQ ID NO: 388 - DNA, 50 bp, Homo sapiens; identical to SEQ ID NO: 209

SEQ ID NO: 389 - DNA, 50 bp, Homo sapiens; identical to SEQ ID NO: 212

SEQ ID NO: 390 - DNA, 50 bp, Homo sapiens
cggtcacgtgataccccccagtgtacctttcctgcagcgtgttacgtggc

SEQ ID NO: 391 - DNA, 50 bp, Homo sapiens
ctggggctgagaccccatttctgggaggctcttcccagtgctggagaccg

SEQ ID NO: 392 - DNA, 50 bp, Homo sapiens
tctttgagccccagcttcctcatgtgtaaaacaggataatagcagtgtcg

SEQ ID NO: 393 - DNA, 50 bp, Homo sapiens
ctgctggggagcagtggacgccctccagggtctagggagcagataagacg

SEQ ID NO: 394 - DNA, 50 bp, Homo sapiens
gcacccccccatccacttcatgttcagaaaactcaaagagtcagaaaacg

SEQ ID NO: 395 - DNA, 50 bp, Homo sapiens
agctctggaatccaactgcctgagtggcaaacctatctgtaagacttacg

SEQ ID NO: 396 - DNA, 50 bp, Homo sapiens
gggcctttagtgctggctcttgagtacccagaccccagttaagaaatacg

SEQ ID NO: 397 - DNA, 50 bp, Homo sapiens
cgacaccctcaagggaggagtgcaggcactcaaagatttgagtcacaggc

SEQ ID NO: 398 - DNA, 50 bp, Homo sapiens; identical to SEQ ID NO: 221

SEQ ID NO: 399 - DNA, 50 bp, Homo sapiens
tggccttaggttctagtggctctggtgtgggcctgtgcccagcctttacg

SEQ ID NO: 400 - DNA, 50 bp, Homo sapiens
tttataaacctgctattcctttccttcggatccctggttttccatctccg

SEQ ID NO: 401 - DNA, 50 bp, Homo sapiens
ctgggcttgacagctcagagcagtgtccccagctgtggccctagaaggcg

SEQ ID NO: 402 - DNA, 50 bp, Homo sapiens
tttgcctctttttcagtcttgtaatcccaaacaaaatagaagagccatcg

SEQ ID NO: 403 - DNA, 50 bp, Homo sapiens
agaagcacgtggcacctgtcataggcccctctggctgctacaagttcccg

SEQ ID NO: 404 - DNA, 50 bp, Homo sapiens
cggcacctatcccagcaagatcccgggaacaaaatcctggaagaccctat

SEQ ID NO: 405 - DNA, 50 bp, Homo sapiens
cgcgtgagtgtcctaaggagtccaagcacaacagatggctgagtcacact

SEQ ID NO: 406 - DNA, 50 bp, Homo sapiens
cgagcctgttgtcaacattagccccgggtttcccagcaccaactccagcg

SEQ ID NO: 407 - DNA, 50 bp, Homo sapiens
cggagcgtgagcctagattctttggaaggctgtacagtttaaaatctaat

SEQ ID NO: 408 - DNA, 50 bp, Homo sapiens
cggcaggttggaaatccagtttgtggctgatgcaagcaaaccatgctgca

SEQ ID NO: 409 - DNA, 50 bp, Homo sapiens
cggttgtgaggtgctcacgtgttttggagatagcaaaagtctcaaataat

SEQ ID NO: 410 - DNA, 50 bp, Homo sapiens
tgtctcctcatctcctggatctttgcccagcaaaacctccaaagagaccg

SEQ ID NO: 411 - DNA, 50 bp, Homo sapiens
cgcacagccagcaggcgcctgggctccactctctacctggaatcaccagg

SEQ ID NO: 412 - DNA, 50 bp, Homo sapiens
cggcagtcttctccactgagggactgggctgggaagtcctgcgtttcagt

SEQ ID NO: 413 - DNA, 50 bp, Homo sapiens
cggccccacccggttcttgtgtcaagacaaaaagaaaacccaggtggcct

SEQ ID NO: 414 - DNA, 50 bp, Homo sapiens
cgctgatagacatcaggtgacaggaaatcagtagcttctgctaccttggg

SEQ ID NO: 415 - DNA, 50 bp, Homo sapiens
cggcaagcatcatcgccaggccccaggcctcctgtgggacgccagtcacc

SEQ ID NO: 416 - DNA, 50 bp, Homo sapiens
cacttcctgactaaggagctgcagcgatacatcgaagggctcaagaagcg

SEQ ID NO: 417 - DNA, 50 bp, Homo sapiens
tccaggaagcagcagaggtcgcgcagctcacggttctctgcctgcagacg

SEQ ID NO: 418 - DNA, 50 bp, Homo sapiens
ccagcttgaagcccggtgccagatgcataagccacttgcccgagagcacg

SEQ ID NO: 419 - DNA, 50 bp, Homo sapiens
cgtagccagtgcgaggttggctctactttgggtttatgggttgggcataa

SEQ ID NO: 420 - DNA, 50 bp, Homo sapiens
cgggcagctctactgcttggagaagagaaagctaggtaactgtacagttg

SEQ ID NO: 421 - DNA, 50 bp, Homo sapiens
cacagccagagcacttacagtgagccgagccacagtccagcaagctgccg

SEQ ID NO: 422 - DNA, 50 bp, Homo sapiens
cgacactgtgataatcatgaagttttgtgtgagaaagataagggagaaga

SEQ ID NO: 423 - DNA, 50 bp, Homo sapiens
atagctattcatccttagaccctgtccaaacagagcaacagtcatatacg

SEQ ID NO: 424 - DNA, 50 bp, Homo sapiens
tatttttgaaggagctggtcagcatttgcctagactctcgggacaacacg

SEQ ID NO: 425 - DNA, 50 bp, Homo sapiens
ccctctagtgagacccattagtgtataagctctgcctacaccgagtttcg

SEQ ID NO: 426 - DNA, 50 bp, Homo sapiens
cggccatgccctggccccagaagtcgttggtgaagatgccccagcagagc

SEQ ID NO: 427 - DNA, 50 bp, Homo sapiens
cggtgatccatagcaaaagagcctatgagtcaggtgatgatccattcatc

SEQ ID NO: 428 - DNA, 50 bp, Homo sapiens
actactttgggcctcggtttccctgctccttgtagatcagagaagggacg

SEQ ID NO: 429 - DNA, 50 bp, Homo sapiens
cggccatgtctggtcactgcgtatgaatgacatctgtctctgcaacgctt

SEQ ID NO: 430 - DNA, 50 bp, Homo sapiens; identical to SEQ ID NO: 242

SEQ ID NO: 431 - DNA, 50 bp, Homo sapiens
cgcagtgacaggaataatgccactgtcctgctgagtgggaaaggagaggg

SEQ ID NO: 432 - DNA, 50 bp, Homo sapiens
agaggtctcaggaaagtagcctttatttatgtggcaccgatcggaacccg

SEQ ID NO: 433 - DNA, 50 bp, Homo sapiens
cgcacagcacggaaagggaaggcagcagccacatggacctgggcccacgg

SEQ ID NO: 434 - DNA, 50 bp, Homo sapiens
cggcaaccccggccagacagggggtatccagagggcccaggacacccacc

SEQ ID NO: 435 - DNA, 50 bp, Homo sapiens
aagaacgactctccgcaatgcgcatgacagaaaagcggctgcttctaccg

SEQ ID NO: 436 - DNA, 50 bp, Homo sapiens
tcgaacgctggacccttgagacatgtgacgggacctgagggcagccaccg

SEQ ID NO: 437 - DNA, 50 bp, Homo sapiens
cggagtttctgttacctgcagggaatgctctcttaactaatccaggggtg

SEQ ID NO: 438 - DNA, 50 bp, Homo sapiens
cggaggctggggagatgacatcagaaaacctggtccaaactgctccaaaa

SEQ ID NO: 439 - DNA, 50 bp, Homo sapiens
ctttactcaatgccaagatccacattaacacaattccactgaatcctccg

SEQ ID NO: 440 - DNA, 50 bp, Homo sapiens; identical to SEQ ID NO: 184

SEQ ID NO: 441 - DNA, 50 bp, Homo sapiens; identical to SEQ ID NO: 186

SEQ ID NO: 442 - DNA, 50 bp, Homo sapiens
ctcttgatgacctcgttgtctgtgctggcaccatgggtctcatcctgacg

SEQ ID NO: 443 - DNA, 50 bp, Homo sapiens; identical to SEQ ID NO: 254

SEQ ID NO: 444 - DNA, 50 bp, Homo sapiens
aagtgtcaacgagatgacttgcgctacagcggcacactggtgaggaaccg

SEQ ID NO: 445 - DNA, 50 bp, Homo sapiens
cgcatctgcttcccatgagtctcttggggaagacaaagctcacattcttc

SEQ ID NO: 446 - DNA, 50 bp, Homo sapiens
ctcagggatctgtgagcagagaggcctggctgcaaagggtctggaggacg

SEQ ID NO: 447 - DNA, 50 bp, Homo sapiens
tgtgacagccctgggctgaaagactcccggtggccgtagtgtaatagccg

SEQ ID NO: 448 - DNA, 50 bp, Homo sapiens
caactgctggtctgttttctgcccctgtagttttgtatgaattctttacg

SEQ ID NO: 449 - DNA, 50 bp, Homo sapiens
cgcaatgtaaaattatgtccagttgtagatgtgtgtgttggggtttaact

SEQ ID NO: 450 - DNA, 50 bp, Homo sapiens
cgggctggaattgagctcagctaaacaaagtccttcagctttgaagggag

SEQ ID NO: 451 - DNA, 50 bp, Homo sapiens
cggacaagataattatgatataacaaaagcttgtgttatttaaggtgggg

SEQ ID NO: 452 - DNA, 50 bp, Homo sapiens
cgtccctggagcccacgaaaatgtctgcaagatctgcaagggccacctta

SEQ ID NO: 453 - DNA, 50 bp, Homo sapiens
cgtcccgacttcacgcgagggtttatacctgaacagacacagcagggaaa

SEQ ID NO: 454 - DNA, 50 bp, Homo sapiens
cgccctctctgtgtagctggaagagcctgaccactcacgtctctccaggc

SEQ ID NO: 455 - DNA, 50 bp, Homo sapiens
aacagccatgattcctaaatattaaacattttcctcatctgacaggatcg

SEQ ID NO: 456 - DNA, 50 bp, Homo sapiens
acagagacagagcccaagaatagaggcacacggggaagtagacaacatcg

SEQ ID NO: 457 - DNA, 50 bp, Homo sapiens
cgagggtagttggtcagagttgtgcgagctggttgcagggaaggctaccg

SEQ ID NO: 458 - DNA, 50 bp, Homo sapiens
caagctctgtgcaaaataatctgtagtgcttgctataacgagctataacg

SEQ ID NO: 459 - DNA, 50 bp, Homo sapiens
cggggataggcaggtaagtaggatcaaggagtgcaaacagccaagtgtga

SEQ ID NO: 460 - DNA, 50 bp, Homo sapiens; identical to SEQ ID NO: 188

SEQ ID NO: 461 - DNA, 50 bp, Homo sapiens
tcggggaagctcagggtcttggggtctcagggcggggaggcaggacgacg

SEQ ID NO: 462 - DNA, 50 bp, Homo sapiens
cgggcagatcccaaggtttcctgatattccctactgctgcagtctctgct

SEQ ID NO: 463 - DNA, 50 bp, Homo sapiens
gtcttcattgttactcagcggggacaccctcctggcgctccgggggctcg

SEQ ID NO: 464 - DNA, 50 bp, Homo sapiens
cgctggagaccaaaatcttgggctatgaccaccctgggcaacatagtgag

SEQ ID NO: 465 - DNA, 50 bp, Homo sapiens; identical to SEQ ID NO: 84

SEQ ID NO: 466 - DNA, 50 bp, Homo sapiens
cgcggcttgactagtaaagtgctcaactattctcgaccaccattgggtat

SEQ ID NO: 467 - DNA, 50 bp, Homo sapiens
atgtggcgggggctttggaccctggcggcccaagcggcacgtgggcctcg

SEQ ID NO: 468 - DNA, 50 bp, Homo sapiens
cggccgccgcccccacccgacccaaccgcccgcacaaaaggccggagccg

SEQ ID NO: 469 - DNA, 50 bp, Homo sapiens
cgggctcggtccagactgacaacaatgccctcctcgtacctgaagaactt

SEQ ID NO: 470 - DNA, 50 bp, Homo sapiens
acgaaggacagtgatccctaacagttcagcagtccctactgtggcaaccg

SEQ ID NO: 471 - DNA, 50 bp, Homo sapiens; identical to SEQ ID NO: 101

SEQ ID NO: 472 - DNA, 50 bp, Homo sapiens
gcacggggcctggcacgtagggggccttcattgcatctctcttcccttcg

SEQ ID NO: 473 - DNA, 50 bp, Homo sapiens
cgggtggggactaaacaaaaaggtcaaggagaaatgtcaacctcaagatg

SEQ ID NO: 474 - DNA, 50 bp, Homo sapiens
cgctgggctctagctctgtatctgtgctcctggcaggccagcaccccatc

SEQ ID NO: 475 - DNA, 50 bp, Homo sapiens
tcaaactgccgcgggcgtgcgggttgacgccgagtgtgtgtgtcggggcg

SEQ ID NO: 476 - DNA, 50 bp, Homo sapiens
ttccagttcgtgccatcaaggagggcgacctgagcaccaagtacgatgcg

SEQ ID NO: 477 - DNA, 50 bp, Homo sapiens
tgagatctctgtctctatcctatcctgtccctggccttctgaggcaagcg

SEQ ID NO: 478 - DNA, 50 bp, Homo sapiens; identical to SEQ ID NO: 190

SEQ ID NO: 479 - DNA, 50 bp, Homo sapiens
tgcatactgatttctgaacattaaatctgcatccaatcgtgtttcatccg

SEQ ID NO: 480 - DNA, 50 bp, Homo sapiens
aaaacaccaacaaaaaacgactcctaacatcactctgggtggtgaaagcg

SEQ ID NO: 481 - DNA, 50 bp, Homo sapiens
cgatccggaattcaggatgagccatgaagttatggatggaggttcgagat

SEQ ID NO: 482 - DNA, 50 bp, Homo sapiens
cgttgttgttgttttagttacgtttagctttgtcagcaacactttggccc

SEQ ID NO: 483 - DNA, 50 bp, Homo sapiens; identical to SEQ ID NO: 352

SEQ ID NO: 484 - DNA, 50 bp, Homo sapiens
cggccagagtcttatcccctggctctggctgatgaggaacacgtagaatg

SEQ ID NO: 485 - DNA, 50 bp, Homo sapiens
cgcggggggtccccctggcacctccaagcccatcccattgacgaagtaac

SEQ ID NO: 486 - DNA, 50 bp, Homo sapiens
cgagagggcagctttaagacattttagaattgtttcttaccattgtcttt

SEQ ID NO: 487 - DNA, 50 bp, Homo sapiens
caagtccagttttccacctaaatatcacttgaggccaacattctctttcg

SEQ ID NO: 488 - DNA, 50 bp, Homo sapiens
cacctgacagacaaagccctgggtccaaaatggctcatcggggtcaggcg

SEQ ID NO: 489 - DNA, 50 bp, Homo sapiens; identical to SEQ ID NO: 361

SEQ ID NO: 490 - DNA, 50 bp, Homo sapiens
tgtgcctccctggcagtcaaagttctaagggggactcctgaagccaggcg

SEQ ID NO: 491 - DNA, 50 bp, Homo sapiens
cggactcgttttattgactgacagtcagtgctagcagtgacttcagctgc

SEQ ID NO: 492 - DNA, 50 bp, Homo sapiens
gtcatagaaggctgtgttgcccccagcaagagcaaagccaccgctccacg

SEQ ID NO: 493 - DNA, 50 bp, Homo sapiens; identical to SEQ ID NO: 200

SEQ ID NO: 494 - DNA, 50 bp, Homo sapiens
gaaaacccagcagaacataaccgtgcaggtctccgacgtcaatgacaacg

SEQ ID NO: 495 - DNA, 50 bp, Homo sapiens
cgcaagagaagaaaaaaggtaagagtttagttctcaaaaagacaaagagt

SEQ ID NO: 496 - DNA, 50 bp, Homo sapiens
cgaaggaaaccttcgctggctccctagtgccctggaataacactgaaacc

SEQ ID NO: 497 - DNA, 50 bp, Homo sapiens
tttaggcaggtggccaattttggtccagctggtggcaagggcaggtgtcg

SEQ ID NO: 498 - DNA, 50 bp, Homo sapiens
cggcaggttttgggactcattcctgcaagcccaagccagaacttgttctg

SEQ ID NO: 499 - DNA, 50 bp, Homo sapiens
cgccattccccagcacccgcagcgggcactgtggctgcacgccgccctcg

SEQ ID NO: 500 - DNA, 50 bp, Homo sapiens
ctgtcagtagatctcagcgggagagcagtgctggtatgtgaatgtcctcg

SEQ ID NO: 501 - DNA, 50 bp, Homo sapiens
cagtcccagctttcactgccagggtcccagtcagattccaggaatttgcg

SEQ ID NO: 502 - DNA, 50 bp, Homo sapiens
cgcccctggagaggcctcttggggaatgaactgtccctcccaaccttgga

SEQ ID NO: 503 - DNA, 50 bp, Homo sapiens
cggcggcaggaactatcagtagacagctgctgcttccatgaaacggaaaa

SEQ ID NO: 504 - DNA, 50 bp, Homo sapiens
cgggccctgcagtccttaataaaaaattgcagatttcattctaggtgtca

SEQ ID NO: 505 - DNA, 50 bp, Homo sapiens; identical to SEQ ID NO: 380

SEQ ID NO: 506 - DNA, 50 bp, Homo sapiens
agatcctaggtgagggcaggttgactggcagggctggtttttcgggatcg

SEQ ID NO: 507 - DNA, 50 bp, Homo sapiens
aaggcctggctggctgcgagctcaggaggccgcctgaggactgcacaccg

SEQ ID NO: 508 - DNA, 50 bp, Homo sapiens; identical to SEQ ID NO: 205

SEQ ID NO: 509 - DNA, 50 bp, Homo sapiens
cggccccacaaattacgtgtgtgcaggattaagggaaaccagcaaggggt

SEQ ID NO: 510 - DNA, 50 bp, Homo sapiens
cgcgccttttattgacgcaaacctcccgttctcgcgggaacttgggaacg

SEQ ID NO: 511 - DNA, 50 bp, Homo sapiens
cgccatcttcacaccccgctccgtcgcgtacgcacctgggtcacgtgata

SEQ ID NO: 512 - DNA, 50 bp, Homo sapiens; identical to SEQ ID NO: 207

SEQ ID NO: 513 - DNA, 50 bp, Homo sapiens
cggccctgcacacgtgtccactgtgacgcgtctgtcatggtcccctcggc

SEQ ID NO: 514 - DNA, 50 bp, Homo sapiens
cggctggggaccgtagcaagagcaagagggctcctcagcagtccctgtgg

SEQ ID NO: 515 - DNA, 50 bp, Homo sapiens
cgccagtatggaaacacagtgtgtaaagcaagcttcgagagaggaaagag

SEQ ID NO: 516 - DNA, 50 bp, Homo sapiens
cgcctacaactctctcggtcaaacaaccgaaaacatcccgtgccggaagc

SEQ ID NO: 517 - DNA, 50 bp, Homo sapiens
ggtgcgccctgggcagctgggtggcctcaagccctactggcgagactccg

SEQ ID NO: 518 - DNA, 50 bp, Homo sapiens; identical to SEQ ID NO: 209

SEQ ID NO: 519 - DNA, 50 bp, Homo sapiens
ggatgcactgcgagcctgccaggaattccaggcctcgcagtgttctggcg

SEQ ID NO: 520 - DNA, 50 bp, Homo sapiens
cgcttccacatttggacgcccccacccagcggcctccgtggcacacaccg

SEQ ID NO: 521 - DNA, 50 bp, Homo sapiens
ggaggacttggggtgtggcaggggagcagccaagccggcagatgactacg

SEQ ID NO: 522 - DNA, 50 bp, Homo sapiens; identical to SEQ ID NO: 300

SEQ ID NO: 523 - DNA, 50 bp, Homo sapiens
acacagaaatgggggttctcacactacagattaaggagtgtcccaggccg

SEQ ID NO: 524 - DNA, 50 bp, Homo sapiens
cgggacaagaaacaacatgtgagcagcacagccattcagttgggatgctg

SEQ ID NO: 525 - DNA, 50 bp, Homo sapiens
ggcgggccttgcctccagcaggggtgtgaagagcccaggcttattttccg

SEQ ID NO: 526 - DNA, 50 bp, Homo sapiens; identical to SEQ ID NO: 301

SEQ ID NO: 527 - DNA, 50 bp, Homo sapiens
tcctgcaggcctcaccatagggcacctctttggcccaattcagggctccg

SEQ ID NO: 528 - DNA, 50 bp, Homo sapiens
ctctgaagcctgcacctctccattaaacacagaacagctgccagaggacg

SEQ ID NO: 529 - DNA, 50 bp, Homo sapiens
cggtgtgagtgctcactcaatgcaatgtgttggtgatggtaactgtcctt

SEQ ID NO: 530 - DNA, 50 bp, Homo sapiens; identical to SEQ ID NO: 302

SEQ ID NO: 531 - DNA, 50 bp, Homo sapiens
cgctgctgcctgggactcagtgattatcccattttgcagaccagaaagag

SEQ ID NO: 532 - DNA, 50 bp, Homo sapiens
agccggacaagtgagaccaggcggccccttgggtgggcagggtctgtccg

SEQ ID NO: 533 - DNA, 50 bp, Homo sapiens
cggctcagcttgctcacccaccccagaaggagcgatttgcatttatgaag

SEQ ID NO: 534 - DNA, 50 bp, Homo sapiens
cgggcaaggaaaggatacaggtatctgcctttcgcatggcactgagcaaa

SEQ ID NO: 535 - DNA, 50 bp, Homo sapiens
cgggacaagcttgacaaggtgggtgtcttcctggactatgaccaaggctt

SEQ ID NO: 536 - DNA, 50 bp, Homo sapiens
cggtagagaatattttgactccttgagtaatgggagttcttttgtggtct

SEQ ID NO: 537 - DNA, 50 bp, Homo sapiens
cgcgctgcagtcacgcctcccgctgccagcccggcaccgggatcttaatc

SEQ ID NO: 538 - DNA, 50 bp, Homo sapiens
ggaggaggatccccgagaggggcgcaagttgcgatgtccggaagccgacg

SEQ ID NO: 539 - DNA, 50 bp, Homo sapiens
cgccagcagatacaaaggcagacaaagtgagcgaggcagtttccaggacc

SEQ ID NO: 540 - DNA, 50 bp, Homo sapiens; identical to SEQ ID NO: 309

SEQ ID NO: 541 - DNA, 50 bp, Homo sapiens; identical to SEQ ID NO: 221

SEQ ID NO: 542 - DNA, 50 bp, Homo sapiens
cgggtggaaggagaatgaggaggcaaccaaaataagatcaaaaagtcagg

SEQ ID NO: 543 - DNA, 50 bp, Homo sapiens
cgatgagcaaaatcacacatcctcatgtccatctggtgctctgtattgtg

SEQ ID NO: 544 - DNA, 50 bp, Homo sapiens
gcggagccagcgctcttgggggcagggctgcgagtcccctgtgtgggacg

SEQ ID NO: 545 - DNA, 50 bp, Homo sapiens
cgtgacctgtctgtaccctagcgcggggcttctgtacgctgctaggaagc

SEQ ID NO: 546 - DNA, 50 bp, Homo sapiens
gaagcagttaagacaacaatacccaggactagccagatcccgaattaccg

SEQ ID NO: 547 - DNA, 50 bp, Homo sapiens
cgtcgggctcacagaaggctcaggtttcctccagtatagttcaggggatg

SEQ ID NO: 548 - DNA, 50 bp, Homo sapiens
cgcctcatacaagaacacagaacagggagcttgtctccttggggattaga

SEQ ID NO: 549 - DNA, 50 bp, Homo sapiens
cgctgcggcaaacctaggagggacccaaaagcagaaaatcctagaaaaga

SEQ ID NO: 550 - DNA, 50 bp, Homo sapiens
cggaaactgatctagtcagggaggtcagagaatatctccctgaggaaaag

SEQ ID NO: 551 - DNA, 50 bp, Homo sapiens
cgcactgactggtgagcgctttgcaccaattagtagcaggtgctacagcc

SEQ ID NO: 552 - DNA, 50 bp, Homo sapiens; identical to SEQ ID NO: 229

SEQ ID NO: 553 - DNA, 50 bp, Homo sapiens
cggggtgcattagctgtgacttttgctgcatccagtcatgcacatgtgcc

SEQ ID NO: 554 - DNA, 50 bp, Homo sapiens
gctttctgctttcaccgggaggccctttaattgttaccaaaaataggacg

SEQ ID NO: 555 - DNA, 50 bp, Homo sapiens
aggtactggatgcacggcaggccctgccactgcttctcagaaccctctcg

SEQ ID NO: 556 - DNA, 50 bp, Homo sapiens
aattctttcacagttctggagtcaagaagtccaaaatgaaggtgttcacg

SEQ ID NO: 557 - DNA, 50 bp, Homo sapiens
cggccctacacgggcaccgggcctcagtcctgccaggcccacgccatcct

SEQ ID NO: 558 - DNA, 50 bp, Homo sapiens; identical to SEQ ID NO: 235

SEQ ID NO: 559 - DNA, 50 bp, Homo sapiens
gaagctggcgacgaacccgtgtctcaagaatttctacggcttgtttcccg

SEQ ID NO: 560 - DNA, 50 bp, Homo sapiens
cggctgcaggccccagagtccacgagggtgggtacaaatcccctgggcac

SEQ ID NO: 561 - DNA, 50 bp, Homo sapiens
tgattggcccaaagcatcgtgaatattcatgacagcagccacaaaggccg

SEQ ID NO: 562 - DNA, 50 bp, Homo sapiens
ttctcgggtcttcgtgagcattaagtcaatgaacccagggcaccaaagcg

SEQ ID NO: 563 - DNA, 50 bp, Homo sapiens
aggccagcgaacatccagctgtcagttggtctggggactatcagcattcg

SEQ ID NO: 564 - DNA, 50 bp, Homo sapiens
gaagatggtgaacctgagatgacctgtcaatgggattcccagacagtccg

SEQ ID NO: 565 - DNA, 50 bp, Homo sapiens
tggataaaggggtttctaatacccagctcacatggctgtggtgacaaacg

SEQ ID NO: 566 - DNA, 50 bp, Homo sapiens
gtgaacacctgccgaagcctttgccttgggagaggctccagcaaaatccg

SEQ ID NO: 567 - DNA, 50 bp, Homo sapiens
cgggcactgactggggacccaggtgagtctagcaaatgacaaggcccaac

SEQ ID NO: 568 - DNA, 50 bp, Homo sapiens
cggcaaggtttataacgagaataaatgaaataaatacaaaatccagaata

SEQ ID NO: 569 - DNA, 50 bp, Homo sapiens
cggggacttgatatggaaagaattaatgtactggcttttttgtatagatg

SEQ ID NO: 570 - DNA, 50 bp, Homo sapiens
cgggtagggttaggctcagttcaggcagaacctgccattcgctcattcac

SEQ ID NO: 571 - DNA, 50 bp, Homo sapiens
attcatctctagtctctgtaaaatgccagccctcttctgggttaacagcg

SEQ ID NO: 572 - DNA, 50 bp, Homo sapiens
cgcaccgtctcacctgagttttctgccactggatcatgtgggtctggttg

SEQ ID NO: 573 - DNA, 50 bp, Homo sapiens
gagtgttccccatgctgacttctgccaggctgcagggaataaagctaacg

SEQ ID NO: 574 - DNA, 50 bp, Homo sapiens
cggaaaggttcattggctaatttgccacagttggttttcaatatgtccat

SEQ ID NO: 575 - DNA, 50 bp, Homo sapiens
ctgtgcagacgccatttgcccccagcttaattgagcatatctctccctcg

SEQ ID NO: 576 - DNA, 50 bp, Homo sapiens
cggtgggaacgggaagcttccccaatcagactgcatcctgagggacagga

SEQ ID NO: 577 - DNA, 50 bp, Homo sapiens; identical to SEQ ID NO: 251

SEQ ID NO: 578 - DNA, 50 bp, Homo sapiens; identical to SEQ ID NO: 253

SEQ ID NO: 579 - DNA, 50 bp, Homo sapiens
cggcctttgtggatgccaacctttgtcacagccaggagggggcctccctc

SEQ ID NO: 580 - DNA, 50 bp, Homo sapiens
cggcctcaggccaagcatgagaacaacgtcagacaaatccccattgattg

SEQ ID NO: 581 - DNA, 50 bp, Homo sapiens
cgccgacccacagggcacaatggtctacaaagttggaaatgaaggtctgc

SEQ ID NO: 582 - DNA, 50 bp, Homo sapiens
gcacgggcagctgagctgggggtacagggcacccccgtgtcccagggtcg

SEQ ID NO: 583 - DNA, 50 bp, Homo sapiens
caggaaactcctacctcatcacggcagctgcatgtgtgggtaagcccacg

SEQ ID NO: 584 - DNA, 50 bp, Homo sapiens
cggcagttcttagtgagggcaattcattcaatccagagccagaaacagga

SEQ ID NO: 585 - DNA, 50 bp, Homo sapiens
cggccacctcagacttctgtataggaggaggcctgactgggagatccctg

SEQ ID NO: 586 - DNA, 50 bp, Homo sapiens
tgtcccaggatgacatcaagggcattcaggagctctatggtaaacctccg

SEQ ID NO: 587 - DNA, 50 bp, Homo sapiens
tatggacagtcttttgcctggcgtgggggccaagtggacaataccacacg

SEQ ID NO: 588 - DNA, 50 bp, Homo sapiens
ctccctccacgggacccagcctgcagaagggtcctgcaggaagtggcacg

SEQ ID NO: 589 - DNA, 50 bp, Homo sapiens
gagtttctactctgcctacaggtctcgggtgaattcacacaaactcttcg

SEQ ID NO: 590 - DNA, 50 bp, Homo sapiens
caagatccagggacctagaggcctcggcgatgacactgcgctgaacgacg

SEQ ID NO: 591 - DNA, 50 bp, Homo sapiens
cgccaatggttccagcaaagccccaggactgctctgctcctggtcttgta

SEQ ID NO: 592 - DNA, 50 bp, Homo sapiens
tcagagctgttttcgtgggtttttaacttccagttgctcaagggtccacg

SEQ ID NO: 593 - DNA, 50 bp, Homo sapiens
cggctccacacttccccagcgtggcctgcatttctattgggcagctggcg

SEQ ID NO: 594 - DNA, 50 bp, Homo sapiens
tatgagaggccagaatattgcttccgttcccttttcatctctgcacaccg

SEQ ID NO: 595 - DNA, 50 bp, Homo sapiens
cgccctgatagcaccgcagaggttctgatctaattgatctgggatgcggc

SEQ ID NO: 596 - DNA, 50 bp, Homo sapiens
atatacagtggccatgaagcaggcaccacttagaaacctctgtattaacg

SEQ ID NO: 597 - DNA, 50 bp, Homo sapiens
cggcagaagcttcaccacaaaagcgaaatgggcacaccacaggtaagact

SEQ ID NO: 598 - DNA, 50 bp, Homo sapiens
cggctagagactcactgactcatgcgtgtgtggtaggaatcttccaggaa

SEQ ID NO: 599 - DNA, 50 bp, Homo sapiens
cgggacggggacttcctggaagattcctaccacacacgcatgagtcagtg

SEQ ID NO: 600 - DNA, 50 bp, Homo sapiens; identical to SEQ ID NO: 188

SEQ ID NO: 601 - DNA, 50 bp, Homo sapiens
ggaaacttgctgtgggtgaccatggcgcacggagccagcgtggatctgcg

SEQ ID NO: 602 - DNA, 50 bp, Homo sapiens
gggtggtacaaggggcgccccttcgctgttttaaaatctgatgcttcacg

SEQ ID NO: 603 - DNA, 50 bp, Homo sapiens
gatttctccttgaacaatccccgcaaagatagcagccaaaaaaggatgcg

SEQ ID NO: 604 - DNA, 50 bp, Homo sapiens
gaaagcactaaattatcctgcaaactcccggctgatgcctaaggaattcg

SEQ ID NO: 605 - DNA, 50 bp, Homo sapiens
cggaagcacagtttgcaacagtttggggttgtcttattttcactgctggc

SEQ ID NO: 606 - DNA, 50 bp, Homo sapiens
cgcacggatgggacctgcttctcactcctgcacagctgaacctccaggac

SEQ ID NO: 607 - DNA, 50 bp, Homo sapiens
ccaggagtgcgctgctctcgggaaggcatcccatggcctgagcagcagcg

SEQ ID NO: 608 - DNA, 50 bp, Homo sapiens
gctgggtccccgtgtagcacttagctaaagatgatcagcagctgagaacg

SEQ ID NO: 609 - DNA, 50 bp, Homo sapiens
acagtatacagtcggtgctcaggatgcatttgttttcctgtcccccagcg

SEQ ID NO: 610 - DNA, 50 bp, Homo sapiens
tgccggccacgtggttgctgggcaggtgtggggtcaggctgtggatcccg

SEQ ID NO: 611 - DNA, 50 bp, Homo sapiens
cggctcagccaaccccctagataatagcggtttctcaaactgtggtcccg

SEQ ID NO: 612 - DNA, 50 bp, Homo sapiens; identical to SEQ ID NO: 268

SEQ ID NO: 613 - DNA, 50 bp, Homo sapiens
cctattcttccagaaccttcctggagtattccgttttctctaggacaacg

SEQ ID NO: 614 - DNA, 50 bp, Homo sapiens
cgggggaattcattgataaggagagcaagcatcccaagaacatccccatc

SEQ ID NO: 615 - DNA, 50 bp, Homo sapiens
cggacacagcaccaggtccagattggcaagaaaggaccctgggcttgctc

SEQ ID NO: 616 - DNA, 50 bp, Homo sapiens
atcttcaagtctcactttggtcctcagtttgtagtatctattgcagaccg

SEQ ID NO: 617 - DNA, 50 bp, Homo sapiens
cggtaccagtaactgccaggaaaaggaagggaatatgtccagaaaaagca

SEQ ID NO: 618 - DNA, 50 bp, Homo sapiens
tggttattccccaggagccgcgcgaagcatgagctaattttcagtgagcg

SEQ ID NO: 619 - DNA, 50 bp, Homo sapiens
cgcacatgaggcacagagaaaggacaaaacgcagccacacctgagctgcg

SEQ ID NO: 620 - DNA, 50 bp, Homo sapiens
gtgcctcccttctgcactgtgggtgtgtggagctgtctttcttggagacg

SEQ ID NO: 621 - DNA, 50 bp, Homo sapiens
tgagcaggagcgagacagagcaccacggggcacgtgaggccagggcaccg

SEQ ID NO: 622 - DNA, 50 bp, Homo sapiens
tcccacagtgaacccctctaggtgcaattacaggatgattttgtgtctcg

SEQ ID NO: 623 - DNA, 50 bp, Homo sapiens
gccccaggaccccgggatgtgcagcctaggggtggggttgaggttctgcg

SEQ ID NO: 624 - DNA, 50 bp, Homo sapiens
acctcttgtggtattcctctatcaggcaatctgggtgggcagagacttcg

SEQ ID NO: 625 - DNA, 50 bp, Homo sapiens
agtcttagcttaaggaaatgtgccacctgcgtgcagggatgaggtcatcg

SEQ ID NO: 626 - DNA, 50 bp, Homo sapiens
ccatgctgcggatcctgtgcctggcactctgcagcctgctgactggcacg

SEQ ID NO: 627 - DNA, 50 bp, Homo sapiens
ttcatcgcaatgggctgtatagcttggcccgtctcattgtaacaaattcg

SEQ ID NO: 628 - DNA, 50 bp, Homo sapiens
tgggctagcccagcgccaccttcctggagactgtctggtggaagacaccg

SEQ ID NO: 629 - DNA, 50 bp, Homo sapiens
cgctgctgaatgcacagcactgtgaatgcacttccatcactgaatataca

SEQ ID NO: 630 - DNA, 50 bp, Homo sapiens
cggggctgagtacttggctgaccaccctagggccacaccagcccagggga

SEQ ID NO: 631 - DNA, 50 bp, Homo sapiens
cgcacaatacgtggaaggccatggaaggcatcttcatcaagcctagtgtg

SEQ ID NO: 632 - DNA, 50 bp, Homo sapiens
aagcacttgatgtttgccctcacactgttcctctcccattccagttgtcg

SEQ ID NO: 633 - DNA, 50 bp, Homo sapiens
ggccttacaccagtgcagagggcaggcttgaggctgatctggtacacacg

SEQ ID NO: 634 - DNA, 50 bp, Homo sapiens
tagaatagtgactggcacataataggtgttcaataaatgtcaacccaccg

SEQ ID NO: 635 - DNA, 50 bp, Homo sapiens
cgcctcagctggtgctccaagacctgctggccagactggtgaggccaggt

SEQ ID NO: 636 - DNA, 50 bp, Homo sapiens
cggggacagggctcctaatgtgtttgtcaagtaaataatgagtaataatc

SEQ ID NO: 637 - DNA, 50 bp, Homo sapiens
cggtgaggccagtgcactcaagtttgggaactaccaatatagagtaaaag

SEQ ID NO: 638 - DNA, 50 bp, Homo sapiens
acatacgtcacattggcagtgtttgtaggatatcgggctgtagggatccg

SEQ ID NO: 639 - DNA, 50 bp, Homo sapiens
gctagctgccgggcattgggagggcttgacgggccagaggtgactgagcg

SEQ ID NO: 640 - DNA, 50 bp, Homo sapiens
cggcacctcgcctcgaccttgccattttatactcaattggggcgtagggt

SEQ ID NO: 641 - DNA, 50 bp, Homo sapiens
gcaggtcattactatgggtaactggggctccatctctctgaaataccacg

SEQ ID NO: 642 - DNA, 50 bp, Homo sapiens
ccctggctggtgtttcatgtccaccagctctgcgttcagcacagcactcg

SEQ ID NO: 643 - DNA, 50 bp, Homo sapiens
cgtctgtcccaaagggcgacacaatcctgaggcagctgttcgcaaactcg

SEQ ID NO: 644 - DNA, 50 bp, Homo sapiens
cggcgcacctctccagtgggacccgcaggacgccgtctctcagccccacg

SEQ ID NO: 645 - DNA, 50 bp, Homo sapiens
taaggcccttcagaaataggatcgacagggctggagtggaggggcccccg

SEQ ID NO: 646 - DNA, 50 bp, Homo sapiens
ctagcatggtgcctaacagctcctaccaaatagtagatgctcagtaaacg

SEQ ID NO: 647 - DNA, 50 bp, Homo sapiens
cggtcagtctgcctacagagtgcttgccaggcaatgaaggaagagcatgc

SEQ ID NO: 648 - DNA, 50 bp, Homo sapiens
cgtgcgaacatgaactaataatccctttgggtgtctggaatgcctgccca

SEQ ID NO: 649 - DNA, 50 bp, Homo sapiens; identical to SEQ ID NO: 199

SEQ ID NO: 650 - DNA, 50 bp, Homo sapiens; identical to SEQ ID NO: 281

SEQ ID NO: 651 - DNA, 50 bp, Homo sapiens
caacactgtgaaaccctgtctctactaaaatacaaaatattagtcagtcg

SEQ ID NO: 652 - DNA, 50 bp, Homo sapiens
cggtagggtttggaggtattattcagtgtagaggaaacagtatgcataaa

SEQ ID NO: 653 - DNA, 50 bp, Homo sapiens
cgctggcaagatgaatcacaataacaactctgaaggcaagaggattggtg

SEQ ID NO: 654 - DNA, 50 bp, Homo sapiens
cggcagaattgtgcttaatagttggtgaggtttctatgggcgatgtggaa

SEQ ID NO: 655 - DNA, 50 bp, Homo sapiens
cttccttcagggagtcgtatatatgagagggctttagcttgctctcctcg

SEQ ID NO: 656 - DNA, 50 bp, Homo sapiens
cgggacacgtactatctgcctcagcctagtgctaagcactttacacattt

SEQ ID NO: 657 - DNA, 50 bp, Homo sapiens
cggggctcatggctaaagttaaggtactgatcaaagttttggatgtaaat

SEQ ID NO: 658 - DNA, 50 bp, Homo sapiens
cgctccaggcagcgctccacttccgcggcttcgcccttgacagcgccctg

SEQ ID NO: 659 - DNA, 50 bp, Homo sapiens
ggagggcatcttattttaccaggtaaacaagggtcactaagaggcatgcg

SEQ ID NO: 660 - DNA, 50 bp, Homo sapiens
ttcacacttagggctcaggacgcccctgtaggcagggtgctggtgggacg

SEQ ID NO: 661 - DNA, 50 bp, Homo sapiens
cgcaaaagcaagattcgctccaggagtttcatgccacaggatggtcgacg

SEQ ID NO: 662 - DNA, 50 bp, Homo sapiens
gctcatcacctgggggcagcttttgtacctgcaccctgtatgaggctccg

SEQ ID NO: 663 - DNA, 50 bp, Homo sapiens
ggtctctggcatctgtcccgtctccagcacaaacaacatctgggcaatcg

SEQ ID NO: 664 - DNA, 50 bp, Homo sapiens
gctgagggtgccaggttgtcctccaaggccatcagaaagaaggcaccacg

SEQ ID NO: 665 - DNA, 50 bp, Homo sapiens; identical to SEQ ID NO: 205

SEQ ID NO: 666 - DNA, 50 bp, Homo sapiens
cagcctcatgaactccatgggtgtcgtcacgctcctcatttggctcttcg

SEQ ID NO: 667 - DNA, 50 bp, Homo sapiens
cgttcagtgccactcaggcctggctgcgaagatacagatggtatatgtga

SEQ ID NO: 668 - DNA, 50 bp, Homo sapiens
ggcagtgttgactgcgttccataccgggacatccaacacaacatttgtcg

SEQ ID NO: 669 - DNA, 50 bp, Homo sapiens
tgattctggacctcagctcttcaacaaagctgaggtccagaatcaaaccg

SEQ ID NO: 670 - DNA, 50 bp, Homo sapiens
agctttctgggtctccttaatgagcctgaggcctgctgcctgcaagtgcg

SEQ ID NO: 671 - DNA, 50 bp, Homo sapiens
cctgaggctctgggagcagatgggagcacaggctctgttttggccctgcg

SEQ ID NO: 672 - DNA, 50 bp, Homo sapiens
tgcaatgataagtttgctgaactgcatctctgcccaatgccacttcctcg

SEQ ID NO: 673 - DNA, 50 bp, Homo sapiens
cccatgcaggagaaacccgtttggtgtttactactaagtcatgatctccg

SEQ ID NO: 674 - DNA, 50 bp, Homo sapiens
cgctgtgtgtgttgagacacacgcaacattcgtgcacatagaactcatga

SEQ ID NO: 675 - DNA, 50 bp, Homo sapiens
cggtgccccacaggccactgtgcaggatctccactcggccctgacacagg

SEQ ID NO: 676 - DNA, 50 bp, Homo sapiens
cgggtccccagtcctcaaggtcccagcacaatgccccaggaggaagactc

SEQ ID NO: 677 - DNA, 50 bp, Homo sapiens
cgccccaagtcatgagggaagcttccagactgactcaggctcaggctggc

SEQ ID NO: 678 - DNA, 50 bp, Homo sapiens
cggtgactgcaggctcctggatcccatggagcagaaacctgaacttgtct

SEQ ID NO: 679 - DNA, 50 bp, Homo sapiens
tggctaccgtgctgtggggtgcctcgaaagtgtgaatcaccaaatattcg

SEQ ID NO: 680 - DNA, 50 bp, Homo sapiens
tgttcaatgtaataaacaactggctctttgctgcttcagatctgtgctcg

SEQ ID NO: 681 - DNA, 50 bp, Homo sapiens
ttatcaaagactttatattttctgtaaaatactacacagtaaatcttccg

SEQ ID NO: 682 - DNA, 50 bp, Homo sapiens
ctaccctactggaaaatagtgttaattattattcagttctatttccatcg

SEQ ID NO: 683 - DNA, 50 bp, Homo sapiens
tcttctttccacaggttctcaggcaagagccacctgctattgccgaaccg

SEQ ID NO: 684 - DNA, 50 bp, Homo sapiens
cgtggctatgctgtggtctccctgagcctactctagctggaaaggtaatt

SEQ ID NO: 685 - DNA, 50 bp, Homo sapiens; identical to SEQ ID NO: 212

SEQ ID NO: 686 - DNA, 50 bp, Homo sapiens
cgacactgcacatcaccgagaccaggcacagtgccggttatgcctaagca

SEQ ID NO: 687 - DNA, 50 bp, Homo sapiens
ctcccgagttcgcccaacttactactctgcatgctggtgcctagtctgcg

SEQ ID NO: 688 - DNA, 50 bp, Homo sapiens
caacggaacgaagctgcatctaagtcttattctagaattctttgtgaccg

SEQ ID NO: 689 - DNA, 50 bp, Homo sapiens
cggacaattggggccaaacgaggaaggacacagacccaaaagccagaccc

SEQ ID NO: 690 - DNA, 50 bp, Homo sapiens; identical to SEQ ID NO: 391

SEQ ID NO: 691 - DNA, 50 bp, Homo sapiens
aacaattatgggcttaaagaattgatcattacagcccctgggatttagcg

SEQ ID NO: 692 - DNA, 50 bp, Homo sapiens
cgccataagtgcccccagaacttcagcgcccaccatggcgcacaaggccg

SEQ ID NO: 693 - DNA, 50 bp, Homo sapiens
cggtgagtcatgcttcaggtttgccagggcctgtgtcccgcaaaaaggcg

SEQ ID NO: 694 - DNA, 50 bp, Homo sapiens
cgctgggaggcaccacttgacatgacctgggacaggtggctcagtctctc

SEQ ID NO: 695 - DNA, 50 bp, Homo sapiens
ctctgcatcctccccaagcaaaacctcaccaaggtggtgagatcctgacg

SEQ ID NO: 696 - DNA, 50 bp, Homo sapiens
cgggggcgccgcctagaaacacacaatggcccctcctggccaaccccccg

SEQ ID NO: 697 - DNA, 50 bp, Homo sapiens
cgcgtcataaaggacaagcagacccaactgaaccgcggctttgccttcat

SEQ ID NO: 698 - DNA, 50 bp, Homo sapiens
caacctcaggttccttttaatggagtagtcacttattcattcaacatacg

SEQ ID NO: 699 - DNA, 50 bp, Homo sapiens
acagtcatactgtcctgagtaaggacagtcaacaaaggatcatttctccg

SEQ ID NO: 700 - DNA, 50 bp, Homo sapiens
cgcgtaacactgtgcctggctttgcaaatatattttacagatagtgtagt

SEQ ID NO: 701 - DNA, 50 bp, Homo sapiens
ctgaccaaggcatcacaataaatacagttagcagcacacagaagcctgcg

SEQ ID NO: 702 - DNA, 50 bp, Homo sapiens
cgacattaaaagaccaatggagaatgtatattagcaatctgtaaggcagt

SEQ ID NO: 703 - DNA, 50 bp, Homo sapiens
cgccgccatctcaggtctcttggctttgccagggcccaccggagaaaact

SEQ ID NO: 704 - DNA, 50 bp, Homo sapiens
gtcagttttctccggtgggccctggcaaagccaagagacctgagatggcg

SEQ ID NO: 705 - DNA, 50 bp, Homo sapiens
gagaggcgcaggcgagctggaggggagcggcgcgcggcggccagtgggcg

SEQ ID NO: 706 - DNA, 50 bp, Homo sapiens
gagagttcaaagtgagcttacttccagtctcacgtacagatgattctacg

SEQ ID NO: 707 - DNA, 50 bp, Homo sapiens
cgggatggaagttagcgaatttgggcaacttgcctctactgcccagtcga

SEQ ID NO: 708 - DNA, 50 bp, Homo sapiens
cgtgggcgagttggtggcaaaatctgaactggatactcacggagggcccg

SEQ ID NO: 709 - DNA, 50 bp, Homo sapiens
ctttggtgcagaaccaccgcatccactttctcaggcccaggggaggggcg

SEQ ID NO: 710 - DNA, 50 bp, Homo sapiens
aagcaggcatggttgatttcccgctagcgggaacgatctggcctcagacg

SEQ ID NO: 711 - DNA, 50 bp, Homo sapiens
cggcagagagttgccactgcaacgcctggctcccagccctcccacccagc

SEQ ID NO: 712 - DNA, 50 bp, Homo sapiens
cgccatctcagccctggtgagccccaaatctgagagggagggaaggtcct

SEQ ID NO: 713 - DNA, 50 bp, Homo sapiens
cgcccccagctgccagtccccagcagctcagtcctgcagtgagagtcttg

SEQ ID NO: 714 - DNA, 50 bp, Homo sapiens
cggaggccaggccacgcagaacctcacagaccaaagctgcttcgcagtcg

SEQ ID NO: 715 - DNA, 50 bp, Homo sapiens
cctgcgggactaccagaaggtgctagtgcagctggagagcctggagaccg

SEQ ID NO: 716 - DNA, 50 bp, Homo sapiens
cggccgggactctccatgtcctatggactctcgctgaagccactcggccc

SEQ ID NO: 717 - DNA, 50 bp, Homo sapiens; identical to SEQ ID NO: 302

SEQ ID NO: 718 - DNA, 50 bp, Homo sapiens
gcggtgtgcactgtgacccgccttcccgggaaagtcagagcacagaagcg

SEQ ID NO: 719 - DNA, 50 bp, Homo sapiens
cgcccctgcctgctcgctgcactccaggtcacagttggcacagcgcaccg

SEQ ID NO: 720 - DNA, 50 bp, Homo sapiens
gaggagtgggtgggagacacgcgtgtccatgccgcgagggtgtgtcgacg

SEQ ID NO: 721 - DNA, 50 bp, Homo sapiens
cgccctcggagcccctgcagtcccctcaccgggcgctcccaaacagcccg

SEQ ID NO: 722 - DNA, 50 bp, Homo sapiens
gccgaatttctgaggtatccgggctctggtggactgaggggggcgacgcg

SEQ ID NO: 723 - DNA, 50 bp, Homo sapiens
cggggagggggtagttgtactctgcttgtacagtccttgagcccagttta

SEQ ID NO: 724 - DNA, 50 bp, Homo sapiens
tcccacttttgtgaaccttgagtttttgaaactttcactgaaaaaaaccg

SEQ ID NO: 725 - DNA, 50 bp, Homo sapiens
cgcaggaggagttgggaggacaaaaggagaaaatgaactagttgggttac

SEQ ID NO: 726 - DNA, 50 bp, Homo sapiens; identical to SEQ ID NO: 545

SEQ ID NO: 727 - DNA, 50 bp, Homo sapiens; identical to SEQ ID NO: 547

SEQ ID NO: 728 - DNA, 50 bp, Homo sapiens
tcttttaacccagctaacacttctgttaatagtgtcttcagccagatgcg

SEQ ID NO: 729 - DNA, 50 bp, Homo sapiens
ggggcaggacatctcccagacagctggggacaccctttccagcgggagcg

SEQ ID NO: 730 - DNA, 50 bp, Homo sapiens
cggtggggacacagaaccaaaccatatcgtttggtattccagaatttctg

SEQ ID NO: 731 - DNA, 50 bp, Homo sapiens
tctttgcaacgtccctcaagcacttaaggagaggcggcagggcccaagcg

SEQ ID NO: 732 - DNA, 50 bp, Homo sapiens
agcaggacaggcacccgctggccgggaggtcattgactggcagaacgacg

SEQ ID NO: 733 - DNA, 50 bp, Homo sapiens
ggaggaggacttgaatacacgcgtcgctgactcaaagatggtcccctccg

SEQ ID NO: 734 - DNA, 50 bp, Homo sapiens
cccggagcagtgggttcctctgccgggccaggagggtgatggagggaccg

SEQ ID NO: 735 - DNA, 50 bp, Homo sapiens
cgcgccggctgacgtcaccctgtgtcgaccagccccctgagcccggaaag

SEQ ID NO: 736 - DNA, 50 bp, Homo sapiens
gaagcacaaaggcgacgtgactcctagaatctgtccagaacccatggtcg

SEQ ID NO: 737 - DNA, 50 bp, Homo sapiens
gtgacagctgagctgagacctcaagacacagtcacctgggccaccttccg

SEQ ID NO: 738 - DNA, 50 bp, Homo sapiens
cttatgcaaatcacttaggtacatgcaaaagtatcccttctcccggagcg

SEQ ID NO: 739 - DNA, 50 bp, Homo sapiens
cgcgccgcatctccgggaacaacagtctccctcccgagcatcacagccag

SEQ ID NO: 740 - DNA, 50 bp, Homo sapiens
cgctcctcctagctagcggccgccgcccgccgccgcctgcgcctccagct

SEQ ID NO: 741 - DNA, 50 bp, Homo sapiens
cggccccagcctgcccagggcccagctgctggagacccgcagctcgtccc

SEQ ID NO: 742 - DNA, 50 bp, Homo sapiens
cggagggctcaggttacaccccataggagggttcaggtgtccccacatct

SEQ ID NO: 743 - DNA, 50 bp, Homo sapiens
ctccagctggcgcactacaaggtaagaactgaccgcctagggttttgtcg

SEQ ID NO: 744 - DNA, 50 bp, Homo sapiens; identical to SEQ ID NO: 563

SEQ ID NO: 745 - DNA, 50 bp, Homo sapiens
cgcgcagttaaaaaagaactcttactttggttggttggaaaagagctgat

SEQ ID NO: 746 - DNA, 50 bp, Homo sapiens
gtcagagttcgggtgtctgtgggtctctgagcctctgctggcagcacccg

SEQ ID NO: 747 - DNA, 50 bp, Homo sapiens
cgcagctcaagaccctggcgcagttccccaacacgctgctgggcaaccct

SEQ ID NO: 748 - DNA, 50 bp, Homo sapiens
cggctggcaggggccctgtgcccccaggtaccccgtacccctgccaaagt

SEQ ID NO: 749 - DNA, 50 bp, Homo sapiens
cgcaagactaggcaacctccagccagtccctgggtcgggcggatcctccc

SEQ ID NO: 750 - DNA, 50 bp, Homo sapiens
aacatgagacaactgaagtgccctggtttatgtgccctgctcctcctccg

SEQ ID NO: 751 - DNA, 50 bp, Homo sapiens
atttcacagataaggaaactgaggcccaagatggcacagtggcctcgacg

SEQ ID NO: 752 - DNA, 50 bp, Homo sapiens
gagacatggcgacggcgaaggtggcagcctggagccttgggctgaggtcg

SEQ ID NO: 753 - DNA, 50 bp, Homo sapiens
cgcccagcccagattttggcagtgccgaagctccacactttcctaagcag

SEQ ID NO: 754 - DNA, 50 bp, Homo sapiens; identical to SEQ ID NO: 246

SEQ ID NO: 755 - DNA, 50 bp, Homo sapiens
attgtctcccaatttcttcgtctgtaaaatggggctggcagcagtgcccg

SEQ ID NO: 756 - DNA, 50 bp, Homo sapiens
cagccactactccagactttgttcctacaactgacgattgccagaatccg

SEQ ID NO: 757 - DNA, 50 bp, Homo sapiens
cggatccgtttgaaacctgtccggtccctgctttctatgccaggcaaaaa

SEQ ID NO: 758 - DNA, 50 bp, Homo sapiens
cgtggggtagggactttcatcaggacatagagtggcagtcatgtgcttcg

SEQ ID NO: 759 - DNA, 50 bp, Homo sapiens
agtgtccgagtaagcctaatgacacacattcacataactaagaagacacg

SEQ ID NO: 760 - DNA, 50 bp, Homo sapiens
agtccacgtgtcagaggtgtttgaaccagagcaaccctatcttaaatacg

SEQ ID NO: 761 - DNA, 50 bp, Homo sapiens
actttctccttcttgtttttattcggcatggctggagcgggccgccgccg

SEQ ID NO: 762 - DNA, 50 bp, Homo sapiens
cgcagagagatgtaccaacactgtgctcctgagtgacttataaagagcca

SEQ ID NO: 763 - DNA, 50 bp, Homo sapiens
tttaagttaaaattgcccagacgtggtattctgaatctgggtgattggcg

SEQ ID NO: 764 - DNA, 50 bp, Homo sapiens
cgctcctggttgtcacattctggctcttttatggggtgggaaatctttca

SEQ ID NO: 765 - DNA, 50 bp, Homo sapiens
cgctgccaggaggagccgaggcgagtgggcgtggctctggcgagtgcccg

SEQ ID NO: 766 - DNA, 50 bp, Homo sapiens
cgccagccccaagcaagccaggcagtgtcctggtgtggcagctcacaggc

SEQ ID NO: 767 - DNA, 50 bp, Homo sapiens
tcatccaggctgcagtgcaatggagcgatcttggcttaccataacttccg

SEQ ID NO: 768 - DNA, 50 bp, Homo sapiens
gtggtggagatgcctgacatggcttggggacctgctgccgggggagctcg

SEQ ID NO: 769 - DNA, 50 bp, Homo sapiens
gtgcagggggagctggcgcagctcaaggcctgggtgaggaagctgcagcg

SEQ ID NO: 770 - DNA, 50 bp, Homo sapiens
cggggctctcccagatgcccacgctgcctgctcccactggagacggggac

SEQ ID NO: 771 - DNA, 50 bp, Homo sapiens
aattggaatgtggcagggaaacgctgggagacccctccccatccttctcg

SEQ ID NO: 772 - DNA, 50 bp, Homo sapiens
cggcaacatcactccagagagcccagcagcttcctgggagaggcaggctg

SEQ ID NO: 773 - DNA, 50 bp, Homo sapiens
gagggtcaggtctgtgctgggggtgaggtccatgctgggggtcaggtccg

SEQ ID NO: 774 - DNA, 50 bp, Homo sapiens
gtctggtcaagagagatccagacaaaatcaaccttctgcgtcaacagccg

SEQ ID NO: 775 - DNA, 50 bp, Homo sapiens
cgcagggcactcggagcaggtctctggctgcctggcacaggaagggcctc

SEQ ID NO: 776 - DNA, 50 bp, Homo sapiens
cgctgatactgacatttacagatgaaaccgtctgagacccgcttcccagc

SEQ ID NO: 777 - DNA, 50 bp, Homo sapiens
agggtgtcggcagcaagatggctccgggggtttagacactgctggcttcg

SEQ ID NO: 778 - DNA, 50 bp, Homo sapiens
cgcaccccagccagagagggaatactgcacctcccagaatgtggcctggg

SEQ ID NO: 779 - DNA, 50 bp, Homo sapiens
aagtacccctgccgctattgtgagaaagtgtttgctctggcggagtaccg

SEQ ID NO: 780 - DNA, 50 bp, Homo sapiens
tcaggagaaatttctaactgtaaccaaagggagcaggcaggacccagacg

SEQ ID NO: 781 - DNA, 50 bp, Homo sapiens
cgcggctcaaccaagcctagaagtgggggcggggaatcttccgccctcct

SEQ ID NO: 782 - DNA, 50 bp, Homo sapiens
cggtattgtcatgttgcatcaaggttcctcattgcagacagaaatctgcc

SEQ ID NO: 783 - DNA, 50 bp, Homo sapiens; identical to SEQ ID NO: 597

SEQ ID NO: 784 - DNA, 50 bp, Homo sapiens; identical to SEQ ID NO: 188

SEQ ID NO: 785 - DNA, 50 bp, Homo sapiens
agctgaaggtcttgaggcgcaggctggtgtccagggggcggctcatcccg

SEQ ID NO: 786 - DNA, 50 bp, Homo sapiens; identical to SEQ ID NO: 601

SEQ ID NO: 787 - DNA, 50 bp, Homo sapiens
cgcacccagccctttacaagcagcacaaacgtatttggttgtctggggcc

SEQ ID NO: 788 - DNA, 50 bp, Homo sapiens
caggaggcatgtgggggcctctgccaggcactgcacaggagggcgcgtcg

SEQ ID NO: 789 - DNA, 50 bp, Homo sapiens
gcctcgcgggattaggggccggtagaggtgggcgggtcgggcggaagtcg

SEQ ID NO: 790 - DNA, 50 bp, Homo sapiens
cgccgaggcccgctgcccgcccccgcccgcccccgcccgcccgcctcacc

SEQ ID NO: 791 - DNA, 50 bp, Homo sapiens
cgcccggctggctagaccattgctaatggctcaagagttcagttctagca

SEQ ID NO: 792 - DNA, 50 bp, Homo sapiens
cgcctgcaattaaaggccagattggaggcatctgatccccagccctgatt

SEQ ID NO: 793 - DNA, 50 bp, Homo sapiens
tgttggacctctaaacggtaattacgggcgacaacgcagatccaggatcg

SEQ ID NO: 794 - DNA, 50 bp, Homo sapiens
gagcagcagcagcatgtacctggccatgctggacggagatgctttgaacg

SEQ ID NO: 795 - DNA, 50 bp, Homo sapiens
gcagccgcagagacccttgggaagtgtggtcttcgggtgccggcggttcg

SEQ ID NO: 796 - DNA, 50 bp, Homo sapiens
cggaagggatgttgttttgcttccgcagacacctgacctccaacttccta

SEQ ID NO: 797 - DNA, 50 bp, Homo sapiens
cgggaatggtgctgtctgcccagccccacccggccttgtaatgaacactt

SEQ ID NO: 798 - DNA, 50 bp, Homo sapiens
tgcctgcaaactaaggcagcattattcagacctgggctaccctggtcccg

SEQ ID NO: 799 - DNA, 50 bp, Homo sapiens
cggtctggttagaaaatatccagccccacagcaaggggaaagagtaacat

SEQ ID NO: 800 - DNA, 50 bp, Homo sapiens
cggatttctgaaaatgtggttattccagagaattccttcacgagatttaa

SEQ ID NO: 801 - DNA, 50 bp, Homo sapiens
cgggtgcttccaaccagtctgctgctcctgccccacccgtgcacgacagc

SEQ ID NO: 802 - DNA, 50 bp, Homo sapiens; identical to SEQ ID NO: 268

SEQ ID NO: 803 - DNA, 50 bp, Homo sapiens
gtgggcgtaggaccgtctgagccatgtgtgggatataatctcctggtgcg

SEQ ID NO: 804 - DNA, 50 bp, Homo sapiens
cgccggaggccgccacaacgcaggcgcattcagctaaggaccactccctc

SEQ ID NO: 805 - DNA, 50 bp, Homo sapiens
cttgtggccatctctgtaaagtttctggggaggtgggcacggggtaaacg

SEQ ID NO: 806 - DNA, 50 bp, Homo sapiens
gcatggcaagaagcacccccaacacccagttctcctggagacactgatcg

SEQ ID NO: 807 - DNA, 50 bp, Homo sapiens
caatacaaattaataacaaccagccaattccattgtccttgtatgcatcg

SEQ ID NO: 808 - DNA, 50 bp, Homo sapiens
cgcgggcaggtgctgctggtgggcgagctgtgggagcgcgaacagagccg

SEQ ID NO: 809 - DNA, 50 bp, Homo sapiens
cgggacagcatgtcactccgggaagcctcccgttcaggtgtctggtccct

SEQ ID NO: 810 - DNA, 50 bp, Homo sapiens
agccaggaagcagttggcaaaggggcggggtgacgcggtgacgcaatccg

SEQ ID NO: 811 - DNA, 50 bp, Homo sapiens
cggaacatgtttgggtatagggagccatcagactgcagtgcacacctgac

SEQ ID NO: 812 - DNA, 50 bp, Homo sapiens
cggcccctggatcctaattcagaccagcctgcctctggcaataggaaagt

SEQ ID NO: 813 - DNA, 50 bp, Homo sapiens
tctagtgtctctagggccacctcactttcagcagtctgtcccaggtgtcg

SEQ ID NO: 814 - DNA, 50 bp, Homo sapiens
tacatctgctcccctgggctttctcaattcctaaataatgttgctgttcg

SEQ ID NO: 815 - DNA, 50 bp, Homo sapiens
ggaatgggaggaacgcaatgcgtcccgcgcggcgatctgggatagctgcg

SEQ ID NO: 816 - DNA, 50 bp, Homo sapiens
cgggagctgtcaatcacgaacaccagatccaggggcccagtgtgacacct

SEQ ID NO: 817 - DNA, 50 bp, Homo sapiens
cgctctcctagagagggcttctgatttggagctgttgttttggtctgaga

SEQ ID NO: 818 - DNA, 50 bp, Homo sapiens
cgggcccctggggcctcagagggaccccggctgccactgacatatgaaga

SEQ ID NO: 819 - DNA, 50 bp, Homo sapiens
agtggctgcagcatgggtcaaggtcagagaatccgggagccccacagccg

SEQ ID NO: 820 - DNA, 50 bp, Homo sapiens
aagcgtacgctctgtgccagtccttaggtaaaatgttttactttgtgccg

SEQ ID NO: 821 - DNA, 50 bp, Homo sapiens
cgccagcccgcggagccccagtgactcagagccgtggctcccctggcccg

SEQ ID NO: 822 - DNA, 50 bp, Homo sapiens
cggctcaggaccagcaggcatgcctccttggtctcatgttgaccttagag

SEQ ID NO: 823 - DNA, 50 bp, Homo sapiens
cgcgactcacccacggtggccgggcagagcctgcctcgaacccggcttct

SEQ ID NO: 824 - DNA, 50 bp, Homo sapiens
ggaggaggctttctgctggctagtacttttccaactctgacagtggcacg

SEQ ID NO: 825 - DNA, 50 bp, Homo sapiens
gaagcacttggacaggccatcgggccagaagcacctcgcaagggtgtccg

SEQ ID NO: 826 - DNA, 50 bp, Homo sapiens
tacttgctcagggctttcttcccgcgtgtgcttggcgctgctcacaaacg

SEQ ID NO: 827 - DNA, 50 bp, Homo sapiens
agatgcctaattcagccgggagccgcgggccggagctggctgaaggtccg

SEQ ID NO: 828 - DNA, 50 bp, Homo sapiens
cataaaccagatgtttcttaaaatagcccagttaaatccacccttcctcg

SEQ ID NO: 829 - DNA, 50 bp, Homo sapiens
cgggcggggaaagcgaggtttaactaactccgcagctatattcttccgcc

SEQ ID NO: 830 - DNA, 50 bp, Homo sapiens
cgccaccccacactccctgcctggggaagtcggacgccgccccacacccc

SEQ ID NO: 831 - DNA, 50 bp, Homo sapiens
cagagagcaaatccttcttcctgccctaggctgcagtgctcctaacctcg

SEQ ID NO: 832 - DNA, 50 bp, Homo sapiens
taaaccgagttaatcatcggtccatttgaataatcagtcacgtggtggcg

SEQ ID NO: 833 - DNA, 50 bp, Homo sapiens
caagcagccaagctgctccacgattggctgctttagccttacgtgcgtcg

SEQ ID NO: 834 - DNA, 50 bp, Homo sapiens
gcaaaccgtgaatgtggggcagtgtggggccaagcggtgcgcttggtacg

SEQ ID NO: 835 - DNA, 50 bp, Homo sapiens
tttctcgaggcagggggcacggtagcacagggagcttctctttgtgggcg

SEQ ID NO: 836 - DNA, 50 bp, Homo sapiens
cgacagccaccttatgtggaaaatactcgcgccggccgtcattcataatc

SEQ ID NO: 837 - DNA, 50 bp, Homo sapiens
cggctcagagcacaggctcagaaatcagactgcccacgtttgaaagctgg

SEQ ID NO: 838 - DNA, 50 bp, Homo sapiens
ggcggcgctgggcattctctgccatccttaggggtcctccacagcatgcg

SEQ ID NO: 839 - DNA, 50 bp, Homo sapiens
cgcacgaacccttcatcctgctccaaacagaatgagaatgtcatgtcgca

SEQ ID NO: 840 - DNA, 50 bp, Homo sapiens
cgctgcccaagtctcagatattcgatgcctcacattgccaatatggagtc

SEQ ID NO: 841 - DNA, 50 bp, Homo sapiens; identical to SEQ ID NO: 654

SEQ ID NO: 842 - DNA, 50 bp, Homo sapiens
catggatttaatcagtgtactttttaccttcaggctgtaaattagaaacg

SEQ ID NO: 843 - DNA, 50 bp, Homo sapiens
cgagatttttaacctgaaactgaagaatctggtactgtaagtgtaaagaa

SEQ ID NO: 844 - DNA, 50 bp, Homo sapiens
cgccgagggctccaggcctcgcttccagccatataggtagtaggccgaga

SEQ ID NO: 845 - DNA, 50 bp, Homo sapiens
cgcctgctctgtgccccactacgcttcatgcaggggtccatgtgcagctc

SEQ ID NO: 846 - DNA, 50 bp, Homo sapiens
cagtaactccggccgaatttgttcgggtgtgaggtttaaggccctaatcg

SEQ ID NO: 847 - DNA, 50 bp, Homo sapiens
gtgactggccaaaaaaaaccgcaattttggggtctaattcgattgtgacg

SEQ ID NO: 848 - DNA, 50 bp, Homo sapiens
gggcggtcaggcggggtcaaggccaggcagcggggcgcgtctgcgttgcg

SEQ ID NO: 849 - DNA, 50 bp, Homo sapiens
ctattggttgagttaaccagcattcaaaagcagtcagcgaaccaactacg

SEQ ID NO: 850 - DNA, 50 bp, Homo sapiens
cggacaggttttaaacaacctaccaagagccagcgtgggtgtccacaccc

SEQ ID NO: 851 - DNA, 50 bp, Homo sapiens
cggggtgaacgtctgggtcctcggaaatcctcagtctctggaactgaatt

SEQ ID NO: 852 - DNA, 50 bp, Homo sapiens; identical to SEQ ID NO: 208

SEQ ID NO: 853 - DNA, 50 bp, Homo sapiens
gggaggccttggttggagtgtctgaggcctcagctgggcccctgcctccg

SEQ ID NO: 854 - DNA, 50 bp, Homo sapiens
cgcagcagccagctcatgggccccgcatccaggtgtgtcctgccctcttc

SEQ ID NO: 855 - DNA, 50 bp, Homo sapiens
cgctgggcactgccctgggggctgagcagctgtctccattggtcattcag

SEQ ID NO: 856 - DNA, 50 bp, Homo sapiens
cggaactcgctggaagctgtgatagtcccagctatggtttatcacaggga

SEQ ID NO: 857 - DNA, 50 bp, Homo sapiens
gagctgcagctggggactggtgcgccatgcaattgacatagcgctgctcg

SEQ ID NO: 858 - DNA, 50 bp, Homo sapiens
tacttcagggtaaagaagttcaggtctgccatctccagctctgtctggcg

SEQ ID NO: 859 - DNA, 50 bp, Homo sapiens
cggcggcttccccaggtgctgctccgcccagtgcccccccagatctcaac

SEQ ID NO: 860 - DNA, 50 bp, Homo sapiens
agcatgaccagaatggttcctcagaatcaggaggtgaaacctaacattcg

SEQ ID NO: 861 - DNA, 50 bp, Homo sapiens
agagtggcgcgagcctgcgttttccggccagaggacatggtgcgttttcg

SEQ ID NO: 862 - DNA, 50 bp, Homo sapiens
ggatcccaaataacagatctgggagaatcctgcctcagtacttggatgcg

SEQ ID NO: 863 - DNA, 50 bp, Homo sapiens
cgcccacagggcccagtgggctctgagtaaggtgcacggcacacaccagc

SEQ ID NO: 864 - DNA, 50 bp, Homo sapiens
gcctgggatcatccccaagtgggtctagggtgggcctgtgaggaggagcg

SEQ ID NO: 865 - DNA, 50 bp, Homo sapiens
cgactgcaggcctacggcttcctttgagggctcacgtttacaagataaca

SEQ ID NO: 866 - DNA, 50 bp, Homo sapiens
cggccgccaaccgaccactgactgtctgccaggcatccgggctccctcca

SEQ ID NO: 867 - DNA, 50 bp, Homo sapiens
ggcctccagagctgggtaagtggagggctctgtgtatgttgctgtacacg

SEQ ID NO: 868 - DNA, 50 bp, Homo sapiens
cgcccatgcccgcgctagtgggaggaggctggaaagcgccttcccatttt

SEQ ID NO: 869 - DNA, 50 bp, Homo sapiens
cgggcagatacgagcagattgactcgccaggactgtcattgggccaccgc

SEQ ID NO: 870 - DNA, 50 bp, Homo sapiens
cggcgctgacgccgcaaggccacttctatcgctcccgaccacggtctgtt

SEQ ID NO: 871 - DNA, 50 bp, Homo sapiens
cgcttgtcagagtcaccatctactaccatgtatttcaggcatggggcaaa

SEQ ID NO: 872 - DNA, 50 bp, Homo sapiens
cgaggtgctggtgttcatacagataaggctctcttcattgcaacagccac

SEQ ID NO: 873 - DNA, 50 bp, Homo sapiens
tcatttgcaaatgttactgggggacacaccggctcccagtagggtttccg

SEQ ID NO: 874 - DNA, 50 bp, Homo sapiens
cgcaagagaagagggagcacgcccagaagctgataatgctgcagaacctg

SEQ ID NO: 875 - DNA, 50 bp, Homo sapiens
cgctgtggcagcccaaacgtcagaggcacctcactttgccatggcctggc

SEQ ID NO: 876 - DNA, 50 bp, Homo sapiens
cggcccagtgaacctgagctttggagtttggacgaatagctagtttacct

SEQ ID NO: 877 - DNA, 50 bp, Homo sapiens
cagggactgacgcccctctagcaaagcatctgtggtacatcccagacccg

SEQ ID NO: 878 - DNA, 50 bp, Homo sapiens
gatctcacactttggagacatacccctaagtagaccagaggcatcacacg

SEQ ID NO: 879 - DNA, 50 bp, Homo sapiens
cgcctggagaagcagtgccaagtctattccctaataaagtacttgttgtg

SEQ ID NO: 880 - DNA, 50 bp, Homo sapiens
cggagctgcagaaagaaagggaagaaactaacgttctttctgcgtctggg

SEQ ID NO: 881 - DNA, 50 bp, Homo sapiens
cgctaaaactcacagcctgtggacaaagcctttttggttttcaaatcggc

SEQ ID NO: 882 - DNA, 50 bp, Homo sapiens
cggtcaaaattaaaaacttctgcactgaaaagaaaaaagggagagagaga

SEQ ID NO: 883 - DNA, 50 bp, Homo sapiens
cgcccccaagaagctccccacccccaaaccagaactggtggctggtgact

SEQ ID NO: 884 - DNA, 50 bp, Homo sapiens
attgaatgccaaagttactggtccccaggcagcagctagcacattcaacg

SEQ ID NO: 885 - DNA, 50 bp, Homo sapiens
cgagtggctactgtattgaacaacacagatctagaaacagagtgtggacc

SEQ ID NO: 886 - DNA, 50 bp, Homo sapiens
cgggaacctccacaggctaaggtgagtgccagcactggcaccagccctgg

SEQ ID NO: 887 - DNA, 50 bp, Homo sapiens
caaaggcagacatcgcttcaggtaggttgcagccaaaatggcttccaacg

SEQ ID NO: 888 - DNA, 50 bp, Homo sapiens
ttctttgtggccaagaaattcccaccttaccacttacagggaggccatcg

SEQ ID NO: 889 - DNA, 50 bp, Homo sapiens
cgcagtgtgaaagatgcgagccatagcatctcgtaacatgaaggccatcc

SEQ ID NO: 890 - DNA, 50 bp, Homo sapiens
tattttgtatttggcttgctctggtttctgctggagcttttaaaaaatcg

SEQ ID NO: 891 - DNA, 50 bp, Homo sapiens
cgggattacctagtgccttcacaatcggtcagagctggattcagattcct

SEQ ID NO: 892 - DNA, 50 bp, Homo sapiens
cgggttactactgtacctaccagctgattccagcagccttttctccagcg

SEQ ID NO: 893 - DNA, 50 bp, Homo sapiens
accgttttttcccccgaataaagtgtgcccgtgtagctgtacagatttcg

SEQ ID NO: 894 - DNA, 50 bp, Homo sapiens
tctttcttcacgtcttgttggttactgctacctggcttccaactgttgcg

SEQ ID NO: 895 - DNA, 50 bp, Homo sapiens
agctggccagactgctgcagttttcagtcccaggaactgagaacgtggcg

SEQ ID NO: 896 - DNA, 50 bp, Homo sapiens
ggatttggtctaggctttctggcttggccctggaactctcagcaaggacg

SEQ ID NO: 897 - DNA, 50 bp, Homo sapiens
cgcaggttacttcctataaatggaagaacctgaatcattaaaagataaaa

SEQ ID NO: 898 - DNA, 50 bp, Homo sapiens
taaggcctcggccatgactgtgggtgggtttaactcagctagcagctgcg

SEQ ID NO: 899 - DNA, 50 bp, Homo sapiens
cgagactaagaagtgacccaacctaggtgacccttcagctaggtcactct

SEQ ID NO: 900 - DNA, 50 bp, Homo sapiens
cgcccataaggatataagggagacagagggaaaaaggaggaagctcactc

SEQ ID NO: 901 - DNA, 50 bp, Homo sapiens
gcaggcgggcctcaggggctgtctttcctgcacggctgttgtgtgcttcg

SEQ ID NO: 902 - DNA, 50 bp, Homo sapiens
cggcaccacacagctagtgccggaactttttgtgcagagaaagaagaccc

SEQ ID NO: 903 - DNA, 50 bp, Homo sapiens
ggtagggtggggccaggctgagcctgctctgcgggtcccggaccccagcg

SEQ ID NO: 904 - DNA, 50 bp, Homo sapiens
cgtgcaggccacagtaatggtggtgcaggtggcaggagtaggtgccctcg

SEQ ID NO: 905 - DNA, 50 bp, Homo sapiens
ggacctgaagatctgcatgtatgaccggctctaccaggactctgtgctcg

SEQ ID NO: 906 - DNA, 50 bp, Homo sapiens
tgacactgtcttcggggcacatatggtcatctatgagtgctgtgagcacg

SEQ ID NO: 907 - DNA, 50 bp, Homo sapiens
gaggggctggcccccttcaccctgtgatcgacaggacagagctgggcacg

SEQ ID NO: 908 - DNA, 50 bp, Homo sapiens
atgcatgtttcacaccttctagaactcagagtaaacctagctcttcaacg

SEQ ID NO: 909 - DNA, 50 bp, Homo sapiens
gttaacaactgtcaacagcctatagaagatcaaggctaaattccctaacg

SEQ ID NO: 910 - DNA, 50 bp, Homo sapiens
cgagtttagcttttaaagaatcctttgaagaaggattgcaacgtgactaa

SEQ ID NO: 911 - DNA, 50 bp, Homo sapiens
tagagaaatacattgtaacaatttggtttctttcctgatggcctttatcg

SEQ ID NO: 912 - DNA, 50 bp, Homo sapiens
attacaagcatgagccagggcacccagccagaaatgatatttaaactacg

SEQ ID NO: 913 - DNA, 50 bp, Homo sapiens
ccatgtataagtccccaggactcacaaatctcctctttcaggatatctcg

SEQ ID NO: 914 - DNA, 50 bp, Homo sapiens
cgttaggtcccacggcttgccctgctcagcacctaataaggccattagct

SEQ ID NO: 915 - DNA, 50 bp, Homo sapiens
cgggggctaagccagcgccgtctgcctctccacctagaccagaccccttc

SEQ ID NO: 916 - DNA, 50 bp, Homo sapiens
cggggggtgccaaaaagccctccttctgacggccctcctggagcccaaca

SEQ ID NO: 917 - DNA, 50 bp, Homo sapiens
cgctttacggaaagaacgccccgcgaataaatccggagcggatttgcatc

SEQ ID NO: 918 - DNA, 50 bp, Homo sapiens
cggagccacagagaacacttttgagaccagcagacaaccacagatgtgcg

SEQ ID NO: 919 - DNA, 50 bp, Homo sapiens; identical to SEQ ID NO: 539

SEQ ID NO: 920 - DNA, 50 bp, Homo sapiens
ttcctatcacaatttacaaaaagcctccaaaaaaccttgaaaagcttacg

SEQ ID NO: 921 - DNA, 50 bp, Homo sapiens
caagggaagctcccgcctcagggtctctgtcttcctgtggttaagagacg

SEQ ID NO: 922 - DNA, 50 bp, Homo sapiens
cgctccggctggtaatttccaaacacagagggaagagcatggtggagcaa

SEQ ID NO: 923 - DNA, 50 bp, Homo sapiens
cggaactgtcctcgacccgtgggtacagtattttctcgtatgccaccaag

SEQ ID NO: 924 - DNA, 50 bp, Homo sapiens
ttggtgcagttttgagcgtccgtgtataaggagtggctccgtagtcaccg

SEQ ID NO: 925 - DNA, 50 bp, Homo sapiens
ccatcagtagagcaggagtcgttggctcaatgcagtgctgtctgcaaccg

SEQ ID NO: 926 - DNA, 50 bp, Homo sapiens
cagtgttcggcagaggacaatctgttcgagaataattagattccccctcg

SEQ ID NO: 927 - DNA, 50 bp, Homo sapiens
cggatgcttaattacaaaaggttttgcccctgtagtgaccgggcagcaat

SEQ ID NO: 928 - DNA, 50 bp, Homo sapiens
cagctcccacctgtgcagagtggcggcctgggagctgagcgtggccctcg

SEQ ID NO: 929 - DNA, 50 bp, Homo sapiens
cgcgcagcttccttacaggaggctttgaatgctgcctggagtatatttga

SEQ ID NO: 930 - DNA, 50 bp, Homo sapiens
cgcttaacaatgagcggggctatatgtcttgcgcttgctctgaaggaagg

SEQ ID NO: 931 - DNA, 50 bp, Homo sapiens
cgccgggagctgctcgcccagtgtcagcagagcctggcccaggccatgac

SEQ ID NO: 932 - DNA, 50 bp, Homo sapiens
cgggtgagtgtttaactttcagcccagcttaagatctccgaagacaccca

SEQ ID NO: 933 - DNA, 50 bp, Homo sapiens
gcagcgtgcctacgctttgttgcaggagcaggttggagggacgctggacg

SEQ ID NO: 934 - DNA, 50 bp, Homo sapiens
aggatgttcagtgactgcagccaggcctacctggagagctttttggagcg

SEQ ID NO: 935 - DNA, 50 bp, Homo sapiens
cggcttctgaactttgtactttgcgagtgtactttgtactttggtcctgt

SEQ ID NO: 936 - DNA, 50 bp, Homo sapiens
cggcctcttatctcgacaatcggttgctcttggccagcccgtcctgctgc

SEQ ID NO: 937 - DNA, 50 bp, Homo sapiens
cgcttatgcccagctgctccagctggaaaagacaggactgcaagtgggtt

SEQ ID NO: 938 - DNA, 50 bp, Homo sapiens
cggactttctgcgcagagaaaacactatctcctttggaggctgtgcactt

SEQ ID NO: 939 - DNA, 50 bp, Homo sapiens
cgctgattgcactgtcaagaaggaaaatactgtttgaaaagacaacagga

SEQ ID NO: 940 - DNA, 50 bp, Homo sapiens
aacaaaccattacgtgttccaattagagcggcagcggacctggctggccg

SEQ ID NO: 941 - DNA, 50 bp, Homo sapiens
cggcagtgagtcacttacatagatgtgtgtaacatgccccagagacctca

SEQ ID NO: 942 - DNA, 50 bp, Homo sapiens; identical to SEQ ID NO: 563

SEQ ID NO: 943 - DNA, 50 bp, Homo sapiens
agcgacacttatgtcctcaatttattgctacgttcactcggtcagagtcg

SEQ ID NO: 944 - DNA, 50 bp, Homo sapiens
ttcatgccggacaaatttccctatgaacaatgcagccaagggctgcatcg

SEQ ID NO: 945 - DNA, 50 bp, Homo sapiens
cgtgggcagagtggttggctgccccactgtcagcctgttctgaaagtagg

SEQ ID NO: 946 - DNA, 50 bp, Homo sapiens
tgcagttcttataataaacacttaaacagggccaggcactgcagttcacg

SEQ ID NO: 947 - DNA, 50 bp, Homo sapiens
aggactagatgttcaccttaaatccagccactgctccagactgcaaatcg

SEQ ID NO: 948 - DNA, 50 bp, Homo sapiens
cgcccttttccggtgtcctgggctcaacagggataaaaggaggcagcact

SEQ ID NO: 949 - DNA, 50 bp, Homo sapiens
ggtggggactggcattaggggtgggcgggagagaccctaaaaatccaccg

SEQ ID NO: 950 - DNA, 50 bp, Homo sapiens
cgtgtgtttgtaattgtgtatggtcctgctaatgtttgtgtttatcactg

SEQ ID NO: 951 - DNA, 50 bp, Homo sapiens
cggttcacagcatgggagcatctgtgctataccaagattactcataggat

SEQ ID NO: 952 - DNA, 50 bp, Homo sapiens
cggggctgtcaagtgtctttaaaaggtcccttcagggtggatggaaacca

SEQ ID NO: 953 - DNA, 50 bp, Homo sapiens
gcccccagctctcaaggccggtgcaaggatgggctgtgctcagcgatgcg

SEQ ID NO: 954 - DNA, 50 bp, Homo sapiens
tcctcagactgttgggatgatgagcggacggtgaactcccaccacctgcg

SEQ ID NO: 955 - DNA, 50 bp, Homo sapiens
agcgggagtcacttcggagtggggtgttgacagcgtgaagcccctgagcg

SEQ ID NO: 956 - DNA, 50 bp, Homo sapiens
cgctttcaggggtcaaagacctggcagaaatgacttcccaaccccagatg

SEQ ID NO: 957 - DNA, 50 bp, Homo sapiens
taattgccctcctgtttcctagaaagcttatagggcagcagtaggaaacg

SEQ ID NO: 958 - DNA, 50 bp, Homo sapiens
cgcagaacagcacagtgtcacatggtcttcacggccctgagggcccaact

SEQ ID NO: 959 - DNA, 50 bp, Homo sapiens
cggggaccaccagctgctttgcccatggattggaacgcattgggtggagt

SEQ ID NO: 960 - DNA, 50 bp, Homo sapiens
gctgttcctcatcactcagtacccagtttgctgacgtctacaatattccg

SEQ ID NO: 961 - DNA, 50 bp, Homo sapiens
cgtgattgcacgtatcaagatgtgtgctcttagatttgttttcaatccag

SEQ ID NO: 962 - DNA, 50 bp, Homo sapiens
cggcgctcagcaaatttagatgaatgcaacgcttcaacgtgggctctcga

SEQ ID NO: 963 - DNA, 50 bp, Homo sapiens
gtcttgatgtgaccagagaacaccatgtacaggcaaagcccagcccctcg

SEQ ID NO: 964 - DNA, 50 bp, Homo sapiens
gctgtcgctgcaggtgggaaccgagagccaggaagcccagggagctgtcg

SEQ ID NO: 965 - DNA, 50 bp, Homo sapiens
acaaggggctcctcctttgtcctgggggagttgcatggatcctgtcttcg

SEQ ID NO: 966 - DNA, 50 bp, Homo sapiens
gttccacatagagagcctggctgcatgatcttgaggtcacctaactcccg

SEQ ID NO: 967 - DNA, 50 bp, Homo sapiens
cgcgcctggcctatacaatattttaaataattttgtgtgtgatacaatga

SEQ ID NO: 968 - DNA, 50 bp, Homo sapiens
cgcccgcctcatttgcgccttgcagcactgctggaccaggtatctgcccg

SEQ ID NO: 969 - DNA, 50 bp, Homo sapiens
cgggtcagaccgtcattggccatctcacagtcccggcgctccagagcccc

SEQ ID NO: 970 - DNA, 50 bp, Homo sapiens
cagccattggctgatttgaaagaatacacagggtgtgccagctggtgtcg

SEQ ID NO: 971 - DNA, 50 bp, Homo sapiens
cggtctcagccgtccccatggtctcagccgtccccagggtctcaggagtc

SEQ ID NO: 972 - DNA, 50 bp, Homo sapiens
cggttatatcaacatgatgcccaaacaccaggtctgcttagggtaaaact

SEQ ID NO: 973 - DNA, 50 bp, Homo sapiens
gtacaaatgggtccaggagcttcaacgagcgttccagcttcttcgtaacg

SEQ ID NO: 974 - DNA, 50 bp, Homo sapiens
cgcgcaccgccccgctccacgcccctatcaggattcgggtcctcgtgagg

SEQ ID NO: 975 - DNA, 50 bp, Homo sapiens
cctcgactgctggctgtgatgttctccaacactgctattcacagcgagcg

SEQ ID NO: 976 - DNA, 50 bp, Homo sapiens
gtcccgttcacactgatcgttccatttcctcttgtgtctgagtgggagcg

SEQ ID NO: 977 - DNA, 50 bp, Homo sapiens
cgggggttggtcagcaccacacactgtgcacagggaagatggagcctcgc

SEQ ID NO: 978 - DNA, 50 bp, Homo sapiens; identical to SEQ ID NO: 776

SEQ ID NO: 979 - DNA, 50 bp, Homo sapiens
tcgatgctggtggtctgcgtggtggttcccaacagcagttcaggggctcg

SEQ ID NO: 980 - DNA, 50 bp, Homo sapiens
ggcggctctagcctctcgggggacgttcggctactccagtggggggttcg

SEQ ID NO: 981 - DNA, 50 bp, Homo sapiens
gaacagccacgcatggtccgtgaaatgggatcatgtgcagaacagccacg

SEQ ID NO: 982 - DNA, 50 bp, Homo sapiens
cgccccaccagcccgagagctagaattgaatctgggggacccctgcggcg

SEQ ID NO: 983 - DNA, 50 bp, Homo sapiens
agcactgtagggagtggccgggatcattcgagcccacagatagtgctccg

SEQ ID NO: 984 - DNA, 50 bp, Homo sapiens
cggacagctaatcgttttagtgacaggatgagagagcccttcgtgttctg

SEQ ID NO: 985 - DNA, 50 bp, Homo sapiens
cggcctgacactctcagagatgggattcccaatccatccactctgaaatg

SEQ ID NO: 986 - DNA, 50 bp, Homo sapiens
ccggaggctgatgccttatccattaggccactgggtcaccacaggatccg

SEQ ID NO: 987 - DNA, 50 bp, Homo sapiens; identical to SEQ ID NO: 785

SEQ ID NO: 988 - DNA, 50 bp, Homo sapiens; identical to SEQ ID NO: 601

SEQ ID NO: 989 - DNA, 50 bp, Homo sapiens
cggcagagaggacaggatcctgccacccagcctcatccccatgcttcccc

SEQ ID NO: 990 - DNA, 50 bp, Homo sapiens
tcccaccttgtgaaactttgccaggtgtcgctcacaggggactgggtccg

SEQ ID NO: 991 - DNA, 50 bp, Homo sapiens
agaacatccactctcttccagccagaataccattaatacgtgtgtcagcg

SEQ ID NO: 992 - DNA, 50 bp, Homo sapiens; identical to SEQ ID NO: 189

SEQ ID NO: 993 - DNA, 50 bp, Homo sapiens
cttcctatgtgattttcttccaacattctcccatgaaaaaatgtcagacg

SEQ ID NO: 994 - DNA, 50 bp, Homo sapiens
tgggtgatggaaactgaggcacagtcatccccccagcaggtccttggacg

SEQ ID NO: 995 - DNA, 50 bp, Homo sapiens
cgggccccccagaatggaacacgagggggtggtctcttgctgggctccag

SEQ ID NO: 996 - DNA, 50 bp, Homo sapiens
cgccagcccagggctggatgttttattttggcatgccccaggtgctcttc

SEQ ID NO: 997 - DNA, 50 bp, Homo sapiens
cgcacatgcgcatccaacccgattccacgggttcccaggaggcggattcc

SEQ ID NO: 998 - DNA, 50 bp, Homo sapiens
cgggaagtctgccagttggcagtctctgacgtaaaagatagcagatactg

SEQ ID NO: 999 - DNA, 50 bp, Homo sapiens
agccccactaatagatattctgattctgttggtctggaatgggaaccgcg

SEQ ID NO: 1000 - DNA, 50 bp, Homo sapiens
ggagggcaggtccgggggctctgtgtccccactgggcccccagcactgcg

SEQ ID NO: 1001 - DNA, 50 bp, Homo sapiens
cattaaagctcagactcgggttttccgagcaggtgttgcaagcctagccg

SEQ ID NO: 1002 - DNA, 50 bp, Homo sapiens
cgggtctctaagatgtcttatgaatgcaggtcagagggtcacatgttaac

SEQ ID NO: 1003 - DNA, 50 bp, Homo sapiens
cagtggatagtgaccaactctgtgttggtcgcctcatgtttcccagcacg

SEQ ID NO: 1004 - DNA, 50 bp, Homo sapiens
agcattcgggcatcagaggtttgtggagagggcagcccagtatacaaccg

SEQ ID NO: 1005 - DNA, 50 bp, Homo sapiens
cgtctaaattacttggagttgatctttctaaacaggattgctcagacaca

SEQ ID NO: 1006 - DNA, 50 bp, Homo sapiens
gcctgaggtcaggagtaagcagacaccagcactgctctttctccaagacg

SEQ ID NO: 1007 - DNA, 50 bp, Homo sapiens
cggaaatcagcttgggggccttctagccctgcagctcagaaaagtgtcag

SEQ ID NO: 1008 - DNA, 50 bp, Homo sapiens
accgcgctcagcccgtggaatttactttataatggggaggcagatgatcg

SEQ ID NO: 1009 - DNA, 50 bp, Homo sapiens
cggttgtcagctgccggaagaagagcgtggaattgagaacacagacccct

SEQ ID NO: 1010 - DNA, 50 bp, Homo sapiens
tgggtgccagggggattatcagcgtctgcgcaaggccgatggtggcagcg

SEQ ID NO: 1011 - DNA, 50 bp, Homo sapiens
tgattggatgcaggattggcgggaaggcagcggggtcatcaaaggctgcg

SEQ ID NO: 1012 - DNA, 50 bp, Homo sapiens
cgatgagctcagccccctcagtccaggccgagagccagatgggggtcacg

SEQ ID NO: 1013 - DNA, 50 bp, Homo sapiens
gtccccctcgtttccttttagaagtcattggccgatcgttttaaaagtcg

SEQ ID NO: 1014 - DNA, 50 bp, Homo sapiens
tgggatcaggatcatggtgagatgtatgcctttcccaggaatgctagccg

SEQ ID NO: 1015 - DNA, 50 bp, Homo sapiens
actactctcctggagtggttacagttaaccaaggcaaaaccccttcttcg

SEQ ID NO: 1016 - DNA, 50 bp, Homo sapiens
cggctgttgtcctgcttacaggactccagagcagcaggaaggagctatgt

SEQ ID NO: 1017 - DNA, 50 bp, Homo sapiens
cgcactcggcctgacccacggcgaccctctgtgaccaatcatactaccaa

SEQ ID NO: 1018 - DNA, 50 bp, Homo sapiens
tattccaatttgggcctgcgtgttcggagctcctggtggcggtctccacg

SEQ ID NO: 1019 - DNA, 50 bp, Homo sapiens
cgggctttggtgaccaggtcttctgtcagtgagcacacatagcccggagg

SEQ ID NO: 1020 - DNA, 50 bp, Homo sapiens
cgcctgtgtggacgcttgtgagctgcaccttcatgctattataatggcga

SEQ ID NO: 1021 - DNA, 50 bp, Homo sapiens
gaaaacacacagatgtcaaaccagaggagctgccaagctgggtaccgacg

SEQ ID NO: 1022 - DNA, 50 bp, Homo sapiens
cgccggccccaggtagtatatttttattggcacaactgccggtatttgcc

SEQ ID NO: 1023 - DNA, 50 bp, Homo sapiens
cggaggatgtgtttccagagagctggtctatttcagactgacaggccact

SEQ ID NO: 1024 - DNA, 50 bp, Homo sapiens
cggcgggactagttcctttgggcataatttaggtgttttgtgaaatgtta

SEQ ID NO: 1025 - DNA, 50 bp, Homo sapiens
tgcttagtagctaaaggccaccttctataacacgaaatagtctacaagcg

SEQ ID NO: 1026 - DNA, 50 bp, Homo sapiens
atgccttcttggggcctggcttgctgctgacgggagcactcaggaatgcg

SEQ ID NO: 1027 - DNA, 50 bp, Homo sapiens
cgacaacagggactcggtggacctggccgagctggtgcccgcggtgggcg

SEQ ID NO: 1028 - DNA, 50 bp, Homo sapiens
acagtcgaagcgcactgctctggtgggggatgttggcggtgcaggaggcg

SEQ ID NO: 1029 - DNA, 50 bp, Homo sapiens
cgaggctaaaatgtggggccagaagataaatctaatgagagctgttgcta

SEQ ID NO: 1030 - DNA, 50 bp, Homo sapiens
cgggggtgtgtttctgtttgtgtaactgggtgtgtgtgtatctagccatc

SEQ ID NO: 1031 - DNA, 50 bp, Homo sapiens
tagaaactgatgttattcatagattccacacattgtatagaagaacatcg

SEQ ID NO: 1032 - DNA, 50 bp, Homo sapiens
cacccccagcctcgccacggctcgctccccccggggtcaggccgttaccg

SEQ ID NO: 1033 - DNA, 50 bp, Homo sapiens
cgggactgtggccaaggccctcagaggccatggggagacacgacaagacc

SEQ ID NO: 1034 - DNA, 50 bp, Homo sapiens
cgcaagcacataacaaaagccaagttaagaaggttagcgatttagttgtc

SEQ ID NO: 1035 - DNA, 50 bp, Homo sapiens
tcaccattgccacttaatggtctgaggggggcttttcctgttactgcacg

SEQ ID NO: 1036 - DNA, 50 bp, Homo sapiens
tggatcgcccaggggcgggcagtccctggaagacaggtacggagtggtcg

SEQ ID NO: 1037 - DNA, 50 bp, Homo sapiens
ggaaacgaatctgggaacgagtttgaagcgcggtcaagtttgactcatcg

SEQ ID NO: 1038 - DNA, 50 bp, Homo sapiens
cgagggtcccagtgttccacatccttgccaacgcctgttattgtctgttg

SEQ ID NO: 1039 - DNA, 50 bp, Homo sapiens
cggggtaaccccaggtcccagtgatttccatagacaaaagagatgctggt

SEQ ID NO: 1040 - DNA, 50 bp, Homo sapiens
agtcttgcctggttacaggcctgtgctctccaggcagaacaagcgcagcg

SEQ ID NO: 1041 - DNA, 50 bp, Homo sapiens
gacagttcttgggaagccggcaaactgcaaaagccccatatttccttccg

SEQ ID NO: 1042 - DNA, 50 bp, Homo sapiens
cgggctcctcaggtctgaggcagctctaccactgacttggtgaattttag

SEQ ID NO: 1043 - DNA, 50 bp, Homo sapiens
cgcctctcaagagcacgatgtaagggctccaagatgagtttgggcttccc

SEQ ID NO: 1044 - DNA, 50 bp, Homo sapiens
ggcacttttcagctctaatgctcttgctttccaaaagcaaaacagaaccg

SEQ ID NO: 1045 - DNA, 50 bp, Homo sapiens
cggggcagcacagacacccgggcaaattcatgatctctaccgagtaaata

SEQ ID NO: 1046 - DNA, 50 bp, Homo sapiens
cgtgtcctttaagaactgtaacactcaccgccagggtccacggcttcatt

SEQ ID NO: 1047 - DNA, 50 bp, Homo sapiens
cgtgaactacccagatgcagcatccgctgttggtgtgatctggaacaccc

SEQ ID NO: 1048 - DNA, 50 bp, Homo sapiens
cggaaggctgaagggggagataatgagctaaagaacaactttcaccaccc

SEQ ID NO: 1049 - DNA, 50 bp, Homo sapiens
tttagtttccttcttttattttcctggcaatagcccaccattgtatatcg

SEQ ID NO: 1050 - DNA, 50 bp, Homo sapiens
cggacactgaggccttgtaatgctgttggctgaagagaggtggttggtca

SEQ ID NO: 1051 - DNA, 50 bp, Homo sapiens
tccgcggggcctgagcagagtcggccttgtaaggcagaggtctcggtgcg

SEQ ID NO: 1052 - DNA, 50 bp, Homo sapiens
cggcctcttgtccaccttgccccgaaggcaagtctggatatgaaaagaaa

SEQ ID NO: 1053 - DNA, 50 bp, Homo sapiens
agcttctttgctttgactgttttcctcttgctgcgtctctttggtcttcg

SEQ ID NO: 1054 - DNA, 50 bp, Homo sapiens
cggattgctgcttctaagcctgagaaggtcatttaatgaactcattgagg

SEQ ID NO: 1055 - DNA, 50 bp, Homo sapiens
cgcgccagcccatgtatgccatggaaatatggctgttggaattctggtgt

SEQ ID NO: 1056 - DNA, 50 bp, Homo sapiens
cgtcttggggacgctatggctccagttctgacactcaagaaacgatggat

SEQ ID NO: 1057 - DNA, 50 bp, Homo sapiens
gggcggcttctgatctcttgcggacagctcagattagtggctcgaggccg

SEQ ID NO: 1058 - DNA, 50 bp, Homo sapiens
cttgggtgcccaggtctcttccttcctgaagaatgcggcacttgcttccg

SEQ ID NO: 1059 - DNA, 50 bp, Homo sapiens
cgggcagactgcgatgaaaccccagtttgttgggatcttgctcagctccc

SEQ ID NO: 1060 - DNA, 50 bp, Homo sapiens
ggtttccaggtagcttgatctgttccaggcctggctggggtctgccctcg

SEQ ID NO: 1061 - DNA, 50 bp, Homo sapiens
acccacctgcccgccggatctggaataatgtgactcgctggtttgtcacg

SEQ ID NO: 1062 - DNA, 50 bp, Homo sapiens
tgctgcggttggagcgctccaccaggatgtccagatgggctttgattgcg

SEQ ID NO: 1063 - DNA, 50 bp, Homo sapiens
ggggtttaaggatgattccccactccacagcctgacgcatcgactctgcg

SEQ ID NO: 1064 - DNA, 50 bp, Homo sapiens
ctacgagtcttatttcctgttaacttttttccttttgcttgatcctatcg

SEQ ID NO: 1065 - DNA, 50 bp, Homo sapiens
cggctgggggaggaggcacccacaagactgccttctaggccacaggccca

SEQ ID NO: 1066 - DNA, 50 bp, Homo sapiens
cggagggagggaggaactgctctggaaatcccctaggccagggcctgctc

SEQ ID NO: 1067 - DNA, 50 bp, Homo sapiens
tgttcctgttactcttcgtgaattttctcaccataaaactgttgccaacg

SEQ ID NO: 1068 - DNA, 50 bp, Homo sapiens
gtactttgatgctctacttggcagaatgtattgcttctggtacccacacg

SEQ ID NO: 1069 - DNA, 50 bp, Homo sapiens
gtgctacctagagaggccagcatgtgggctccacatttctgctgaagacg

SEQ ID NO: 1070 - DNA, 50 bp, Homo sapiens
cggtgcttataatacattcctgtgtgtgtgttcactttgatttacggaaa

SEQ ID NO: 1071 - DNA, 50 bp, Homo sapiens
cgtcaggtttatatctttgggatttgaatgtaaagatgttggattttttt

SEQ ID NO: 1072 - DNA, 50 bp, Homo sapiens
cgctccatgtgacagaaacatgagcgtttccaaaatgaaaacactggggg

SEQ ID NO: 1073 - DNA, 50 bp, Homo sapiens
ttcccttgcttttcccagcttccggtagcccaggcattccttgtcttgcg

SEQ ID NO: 1074 - DNA, 50 bp, Homo sapiens; identical to SEQ ID NO: 208

SEQ ID NO: 1075 - DNA, 50 bp, Homo sapiens
cggctagaggatgacccatcttacgcctatggagaacactgcggaaatca

SEQ ID NO: 1076 - DNA, 50 bp, Homo sapiens
ttgcctgtgtgtgatttatgcatgttcccaccagcaggtgtggattctcg

SEQ ID NO: 1077 - DNA, 50 bp, Homo sapiens
cgggctccgatctccggtgtcacagcaaagatccgcgtctttccgatgaa

SEQ ID NO: 1078 - DNA, 50 bp, Homo sapiens
cgcctccccacgcacttccctgtatgggttacaaagcaggtgcacatcca

SEQ ID NO: 1079 - DNA, 50 bp, Homo sapiens
cgtggcacacagagccaggtttccccgaagtagtctaacgctgttgctaa

SEQ ID NO: 1080 - DNA, 50 bp, Homo sapiens
cattggctcttcacttgttgcttggtgttttccttagtcttctgagatcg

SEQ ID NO: 1081 - DNA, 50 bp, Homo sapiens
cgggacatgaagtctaaggggattattttggagctttaaaacgtgatgac

SEQ ID NO: 1082 - DNA, 50 bp, Homo sapiens
cgggaatttggtgagagtcccccacagttctgtctgccaggcactggcga

SEQ ID NO: 1083 - DNA, 50 bp, Homo sapiens
cgcatcctccagccatgctatgcttgcaaagatgtctctggtcattggga

SEQ ID NO: 1084 - DNA, 50 bp, Homo sapiens; identical to SEQ ID NO: 677

SEQ ID NO: 1085 - DNA, 50 bp, Homo sapiens
ggaagtcctctgtgcatgcgtgtctgtgccataggcgtgggaacacctcg

SEQ ID NO: 1086 - DNA, 50 bp, Homo sapiens
cgcctaggtatgggaaatgtaagtatcctcagcagagaccacagttctct

SEQ ID NO: 1087 - DNA, 50 bp, Homo sapiens
cggtcagcactgggtgaatgggttgagggaacccacataaaatccccaag

SEQ ID NO: 1088 - DNA, 50 bp, Homo sapiens
cgatcttccccatggaagacatgcacatgggttaggagaatacaacactc

SEQ ID NO: 1089 - DNA, 50 bp, Homo sapiens
cgcaacaacttctcagctacagtaaatcaggatttggggtgataggaagg

SEQ ID NO: 1090 - DNA, 50 bp, Homo sapiens
caatgtatactatagcaagtggtaccagtgctgcgggtaccagtgctgcg

SEQ ID NO: 1091 - DNA, 50 bp, Homo sapiens
cacagatcagactgctaagtctttacacatccgaaagttagactttgacg

SEQ ID NO: 1092 - DNA, 50 bp, Homo sapiens
gccacgggagatttcatcagaagaatatcagtctattgatatgggtgccg

SEQ ID NO: 1093 - DNA, 50 bp, Homo sapiens
cctccctacaactgtaggttcccctgctgctgggctcagctgggagctcg

SEQ ID NO: 1094 - DNA, 50 bp, Homo sapiens
cgggacagccccgatgccgatgcctgtgttctgtgtccccaggtctaaag

SEQ ID NO: 1095 - DNA, 50 bp, Homo sapiens
gagcccagcggggttagggttcaggtgagggtttagggtcggggcgagcg

SEQ ID NO: 1096 - DNA, 50 bp, Homo sapiens
cgtaccccgggatctggcatttagctggcaatcaaatatgtggtgaaacg

SEQ ID NO: 1097 - DNA, 50 bp, Homo sapiens
gtttaaaattctctcttctgagtaatagtgttcatgtgctcccattctcg

SEQ ID NO: 1098 - DNA, 50 bp, Homo sapiens
actaggtaaacaccacagtaataactgttgcaggtaagaatcatcaggcg

SEQ ID NO: 1099 - DNA, 50 bp, Homo sapiens
cgggaaatgaccaagcgtctccacaatttaggggcaggtcagggtacctt

SEQ ID NO: 1100 - DNA, 50 bp, Homo sapiens
cgccacaaacccaccaaggtgctctcccccgagtacttgtgggaccagca

SEQ ID NO: 1101 - DNA, 50 bp, Homo sapiens
cggcaccactcatgttcataggccagctgaggctcagggggctgacttcc

SEQ ID NO: 1102 - DNA, 50 bp, Homo sapiens
cgctgggcaaccgtaagtatttagggagacagaggtgcctcttctgcaga

SEQ ID NO: 1103 - DNA, 50 bp, Homo sapiens
cgacgcccttgctcacaggctccattgagaggctgccccggtgctcatct

SEQ ID NO: 1104 - DNA, 50 bp, Homo sapiens
cgcagccctgcgggacctgaaaaggcgagactaagtcaccagccaagctg

SEQ ID NO: 1105 - DNA, 50 bp, Homo sapiens
cggtcactgtttgtcttgaaaaaaagagagaaaatgtttgtcattccagg

SEQ ID NO: 1106 - DNA, 50 bp, Homo sapiens
cgtcttctagcaggtatgagggagacaactacaaacgccagaggctcagc

SEQ ID NO: 1107 - DNA, 50 bp, Homo sapiens
agctctcgccgctgaaggggctcagcctggtcgacaaggtgaacaggccg

SEQ ID NO: 1108 - DNA, 50 bp, Homo sapiens
gcagggcagccagctacgaattttgagctctggggcgcgctcacctggcg

SEQ ID NO: 1109 - DNA, 50 bp, Homo sapiens
cgggtcaagagcagtgacctagtggccctcagccctggatggaggacaga

SEQ ID NO: 1110 - DNA, 50 bp, Homo sapiens
cgccattctgttggtactaaggtgttgtggttggtagaagcttaagtgag

SEQ ID NO: 1111 - DNA, 50 bp, Homo sapiens
cgggtcgtggtgactactaatgggtataagatttctttttgagatgatgg

SEQ ID NO: 1112 - DNA, 50 bp, Homo sapiens
tgttgacctcaggtccagtttgtttgcagcctccctcttctgacagatcg

SEQ ID NO: 1113 - DNA, 50 bp, Homo sapiens; identical to SEQ ID NO: 214